European Patent Application EP 4 696 716 A2, published February 18, 2026. Title: HUMANIZED LIGHT CHAIN MICE. Applicant: REGENERON PHARMACEUTICALS, INC. Application US 13/716238, filed February 15, 2023. The sequence listing filed with the application follows.

SEQUENCE LISTING (200 sequences)

SEQ ID NO: 1 - protein, 754 aa, Mus musculus
MLSLTWGMRLVERPVVPRVLLLLFALWLLLLVPVWCSQGHPTWRYISSEVVIPRKEIYHTKGLQAQRLLSYSLRFRGQRHIIHLRRKTLIWPRHLLLTTQDDQGALQMEYPFFPVDCYYIGYLEGILQSMVTVDTCYGGLSGVIKLDNLTYEIKPLNDSQSFEHLVSQIVSESDDTGPMNAWKHWSHNTGSPSSRLEYADGAPRLSSKNYATHPAAIKGHFQATHSVYSASGGDKLSSTVEYLFKVISLMDTYLTNLHMRYYVFLMTVYTEADPFSQDFRVPGGQAHTFYERVFYAHFRPDAGAIINKNSPGDDAVNPAERSICSPSALICLGQHGRNPLFLSIIITNRVGRSLGLKHDEGYCICQRRNTCIMFKNPQLTDAFSNCSLAEISNILNTPDLMPCLFYDRHVYYNTSLTYKFCGNFKVDNNEQCDCGSQKACYSDPCCGNDCRLTPGSICDKELCCANCTYSPSGTLCRPIQNICDLPEYCSGSKFICPDDTYLQDGTPCSEEGYCYKGNCTDRNIQCMEIFGVSAKNANIKCYDINKQRFRFGHCTRAEESLTFNACADQDKLCGRLQCTNVTNLPFLQEHVSFHQSVISGVTCFGLDEHRGTETADAGLVRHGTPCSRGKFCDRGACNGSLSRLGYDCTPEKCNFRGVCNNRRNCHCHFGWSPPKCKEEGHSGSIDSGSPPVQRRIIKQNLEPVVYLRILFGRIYFLFVALLFGIATRVGVTKIFRFEDLQAALRSWQEQAKDK

SEQ ID NO: 2 - protein, 756 aa, Mus musculus
MLSLTWGMRLVERPVVPRVLLLLFALWLLLLVPVWCSQGHPTWRYISSEVVIPRKEIYHTKGLQAQRLLSYSLHFRGQRHIIHLRRKTLIWPRHLLLTTQDDQGALQMDYPFFPVDCYYIGYLEGIPQSMVTVDTCYGGLSGVMKLDDLTYEIKPLNDSQSFEHLVSQIVSESDDTGPMNAWKHWSHNTGSPSSRLEYADGAPRISSKNYATHPAAIKGHFQATNSVYNSAAGDKLSSTVGYLFQVISLMDTYLTNLHMRYYVFLMTVYTNSDPFRLEFAVPGGSAYNYYVSVFYNKFKPDAGVLLNKYGPQDNQVNPAERSICSSLALICIGKYDRNPLFLSPIITNRVGRSLGLKYDEGYCVCQRRNTCIMFRHPQLTDAFSNCSLAEISNILNTPGLMPCLFYDRHVYYNTSLTYKFCGNFKVDNDEQCDCGSQKACYSDPCCGNDCRLTPGSICDKELCCANCTYSPSGTLCRPIQNICDLPEYCNGTKYICPDDTYLQDGTPCSEDGYCYKGNCTDRNIQCMEIFGVSAKNANIKCYDINKQRFRFGHCTRAEESLTFNACADQDKLCGRLQCTNVTNLPYLQEHVSFHQSIISGFTCFGLDEHRGTETTDAGMVRHGTPCSKSKFCDQGACSGSLSHLGYDCTPEKCSFRGVCNNHRNCHCHFGWKPPECKEEGLSGSIDSGSPPVQRHTIKQKQEPVVYLRILFGRIYFLFVALLFGIATRVGVTKIFRFEDLQATLRSGQGPARDKPK

SEQ ID NO: 3 - DNA, 13894 bp, synthetic construct
  source 1..13894: mol_type = other DNA; note = synthetic
gtcctaaggtagcgagggatgacagattctctgttcagtgcactcagggtctgcctccacgagaatcaccatgccctttctcaagactgtgttctgtgcagtgccctgtcagtggaaatctggagagcatgcttccatgagcttgtgagtagtatatctagtaagccatggctttgtgttaatggtgatgttctacataccagttctctggcttaataatgaggtgatgattctatgttcctgtaacgcttcctcaactgggtcctaagtctttcttcactccatctattcctctaaggaatgatcctgaaaatcccatcacaaactataggagatgggaaccatcaaaaaacacagtgacaaagaggtgggaacgcatcagggttcaggaaccatattttaaaaagatatcgtaaataacttcttaaaagagatatagacaaatctccattaatacggagaccagaggcctaaggctaagaaccaatggtggctcaaggtctcctgctacccgaggagcaaacgtagagcagtttctaatgatttatttaaaatatagaatcaaaagtaccagtttgcaattttgaaagatttatttcagcaatgcaacaacatcaggtggtgccgagtccaacacgtcttatgtcccatgatataaacaaaggccatccagaactgtggactggagttctaccttgtcccctaatgacattcagattttttttccattctctttatcttagaggagacagggggctaactcattttacttgtcctttgcttgttcttgccaagaacgtaaagcagcttgcaagtcttcaaacctaaatatcttagtaactcctacacgagtggcaatgccaaagagcagtgcaacaaagaggaagtaaatacgaccaaagagtattcttaaatacactactggctctaggttctgttttattatgcgcctttgaaccggaggggacccactgtctatgctcccactgtgtccctcttctttgcactttggagggctccaaccaaaatggcaatggcaattccgacgattgttacacactcctctgaaattgcatttttctggggtgcagtcataacccaaacgagataaacttccattgcaagctcctcgatcacagaacttaccccttgaacacggggtaccatgtctcaccaatccagcatctgctgtttctgtcccacgatgttcatcaagcccaaagcaggtaaccccagagataaccgattgatggaatgaaacatgttcttgcaaaaatggaagattggtgacattggtacactgcaaccttccacacagcttgtcctgatcagcacaagcattgaatgtgaggctttcttctgctctagtacaatgcccaaatcgaaaccgttgtttgttgatgtcatagcacttaatattagcattcttagcacttacaccaaagatttccatgcattgtatgttgcgatcagtgcagttacctttatagcagtaaccctcttctgagcatggtgtcccatcttgcagataagtgtcatctgggcaaatgaacttagagccactacagtactctggaagatcacatatgttctggataggtctgcagagtgtcccagaaggactgtaagtgcaatttgcacagcataattctttatcacaaatgctaccaggtgttaacctgcaatcatttccacagcagggatctgaataacatgccttttgggagccacagtcacactgctcattgttatctactttgaagtttccacaaaacttataagtcaatgatgtattataataaacatgacggtcatagaaaagacatggcatcagatcaggagtattaagtatgttgcttatctctgcaagggaacaattgctgaaagcatctgttaattgaggatttttgaacatgatgcaggtgttccttctctggcagatacagtacccctcatcatgttttaggcctaaactccttccaacacgattggttattataatagataaaaataaaggatttcgaccatgttgaccaagacaaattagggctgagggagaacatatactcctctcagctggattaacagcatcatctcctggcgaattcttgttaattatagctcctgcatcaggcctaaaatgagcataaaatactctctcatagaaagtatgagcctgccctcctggaactcgaaaatcttgtgaaaatggatcagcctcggtatacacagtcatgagaaagacatagtaccgcatatgaagattggtcagataggtgtccattaaactaatgactttaaacaaatactcaacagtagatgaaagtttgtcacctccagaagcactatatacagaatgggttgcttgaaagtggccttttatagcagctggatgtgtagcgtaattcttactagatagtctgggagctccatctgcatattccaatctggaggagggagaacctgtattatggctccagtgcttccatgcattcataggccctgtgtcatcagactcagatactatctgagaaacaaggtgttcaaagctctgtgaatcattgaggggtttgatttcataggtaaggttatccaactttatgacccctgacaggcccccataacaagtatccacagtgaccatggattgcaggatcccctccaggtagccaatatagtaacaatctacaggaaaaaaggggtactccatctgtaaggctccttggtcatcttgagttgtcagcaacaagtgtctgggccaaatgagtgtctttctccgcaggtggatgatatgtctctggccccgaaaacgcaagctatacgagagcagtctttgtgcttgaagtcctttggtatggtagatctccttccgaggaataaccacctccgatgagatgtaacgccaagtgggatggccttgagaacaccagactggaaccaggaggagcagccagagtgcaaatagcaagaggaggaccctggggaccacaggtctttccactagcctcatgccccaggtcagagataacatcctgggtggagctaactccctctgctgtggccactgcctggtctagaaaatactgacagaggactaaaaacctcctcaggctcccaacctaagtggttacccagacaactggagttaggtaacagtcactgggtgtggcaggaattgagtctgaatgtgttagctgaggttgaggttaaatattgtcaaaagggatgtctataaatgtgcctggacaagaaaagtcagaagcagcaaggagtgtctctgacaggctcaatcctttcttttctttttttgaagttcaaaatatcatttccacgtgaatgtatttggttcccagtgtgactctgggtctctttctaggagtcaatatttctttatatcttggctcatgtttttcacagttgttctaacttcttgttttgttttgtttgtttgtttgtttgaaagttagaagtaaatactgtctatattagccttttagctataaatgattgtttttatttcttctaatcatgttttgtttgagttttggttaaactatttacaaatgagttttttttttccttttgggtgttgctcgaaagtttggagctttctgttaatattgtgttgttgtttctccaatattattagacctgagaattctacctgggtacctgtgaactccagaatttttaaaaattccatctcttgggaacattatctctgaccccgtctgaggccgaagtggctgtccccctccaacctttagtatctttctttcctgactattgggatttcttcaagcaatcaggctgatgggttctcagcagtgagaccagtagactgtcggtatgaacgtcgaagagtctgccacacactccgggttcatcaacagtgctttcgcgtctcttacttttgtagaaggaaatgcagcctctgagttttctccaagaaatcattgatgaaagggtgaaaagatgggtatcacccggagttcatgacaagccctggctcagacacgtgagcaaggtctacagccccaaagataggctgccctgcaacatgtatttataagataggagaaaaaaatgggtagttggagggttgatcaacttacttcctctcaaacatatatatctcatctaagtgtgcaggggaaaactctgtagaactactgggatacctgctcacccccaggagcctcatgaataagtctctgcttctgccttgtagccatgagcattactgcacctgatacccctgcagcttcctagggaagagggaggaagtgacttggcccctgtctggttaaggtaagaggagataaatcccttctcattgattagggtgagaggggtcatgtgctctatcattggtgacccagttgggacatgggtttataccaaagtcatcactctgaggttctgtgtaccaccaggctgaactcccatatcctacatggacataggacaacaccaagcagaaggaggttttaggactaaactgaaggacagagatgcggtttctaaacaactagggagtgccagggccagcctctctaaccactataggacactgtggagtctggttacaaagagagattactcaaggtccttagcactgattacagagcatatctcagatgccttctgctgaccagatgtatctttgcataatctgcctatccagattcagaaaattgatgccacatagccaagtggactttcaggaacagacgatttaaaaacaggcagagagatgtgagagaaaggagaaggagagagagaagggagagggagagaagagagagggagacggagaaggaaagagggagaaggagaaggagagaaggggcatggacagagggagggacagaaggagagaggagatagagagggggataaggaagaagggagggagggagagagagagaaggctaagtctttccatacctgggtcccaatacctcttataacccaagcacatggtttcacatatcacaatgcggttgggatatagataactgtaaatacttgtgaaaataatggggctgagatctggggttttcatgatagtttcaaagtcaccgtactgactaaaaccttccactggcccatctccagcttcctaatctgagggtatcaaatttcccactaagtgtgtttagaaagatctccacctttttgcccttgtcttccagtgccccacctacgttctggtctcccacatctgatgtcttctcagtgattctggccctgcctgctccacagctacaaaccccttcctataatgagctctgtgctgagccatcatcctgaatcaatccaccttaagcagatgttttgcttatttttcctgtgtccatactacagaggaaaggtaggcatgtagaagctgaagcatctcacctcattccaagcaccctcagtctctaaatgtgcccccttgtttccagaagtgcaacctcaagcatcttttattcattcatcttagagggccacatgtgctgtagtgttataagatgaaatttaaagcattaattattcctaacaagccaattaaacaagccaaaaacattcatcagtcattcccatggaacctctgaagcatcttcctgctctaaccttgggttttccagggctgctctgggatcacaggagctgtcctgtctaccagccatataaaggcagacctatcagaattacaccagacttctcaccatagactataaaagccagaatatcctggacagatgttatacagaaactaagagaacacaaatgccagcccaggctactatacccagcaaaactctcaattaccatcgatgaagaaaccaagatattccattacaagtccaaatttacacaatatctttccataaatccagccctacaaaggatagcagatggaaaactccaacacaggtaggaaaactacaccctagaaagagcactaaagtaatcatctttcaacacactcaaaagaagataaccacacaaacataattccacctctaacaacaaaaataaagtaggcaacaatcactattccttaatatctcttttaacatcaatggactcaattctccaataaaaagacatagactaacagactgaatacataaacaggacacagcattttgctgcataaagcaaacacagcgttacttttttttttctaaatgacattttttattagatattgtctttattgacatttcaaatgttatcccctttcctggtttaccctctgaaatcccctatctcctccccctccccctgctcaccaatccacccactcccacttccaggccctggcaatcccctatatttgggcatagagccttcacaggaccaaggtactctccttgcattgatgaccaactagtccattctctgctacaaatgcagctagatctatgagtcccaccatgttttcttttgttggtggtttcatgccagggagctcttggagtactgattggttcatattgttgttctccctatggggttacaaaacccttcaacttcttgggtcctttctctggctgcctcattggggaccttgtgcgaagtccaatggatgactgtgagcatccacttctgtatttgccaggcactggcagagcctctcagaagacagctatatcaagatcctggcagcaagctcttgttggtatccacaaaagtgtctggtggttgtctatgggatggatccccaaaggggcagtctctggatggtcattccttcagtctctgttccacactttgtctctttaactccttccatgactattttattcctccctctaagaaggaccgaagtattcatactttggtcttccttcttgaaattcatgtgttttgtgaattgtatctttgatattccgaacttctgggctaatatccacttatcagtgagtgaatatcatgtgtgttcttatgtgattgagttacctcactcaggatgatatcctccagaaccatccatttgtctaagaatttaatgaattcattgtttttaatagctgaggagtactccattgtgtaaatgtaccacattttctgtacccattgttctcttgagggacatctgggttctttaaagcttctggacattaaatataaggctgctatggaaatagtggagaatgtgtccttattacatgttggagcatcttctgggtatatgcccaggagtgctattgctggatcctctgatagtactatgtccaattttctgaggaactgccaaactgatttacagagtggttgtaccagcttgcaattccaccagcaatggagaaatgttccccttcctccacatcctcaccaacatctgctgtcacctcaatttgttcttagtgattcagacaggtgtgaggtggaatatcagggttgtttggcatttccctgatgactagtgatattgaaaaaaattttaagtgtttctcagccattcagtattcttcagttgagaattcactgtttagctctgtactcaggtttttttaatagggttatttggttttctggagtctaacgtcttgaattctttctatatattggatattagccctctgtcatatttaggattggtaaagatctttcccaatatgttggctgcctttttgtgtcctttgccttacagaacctttttaattttatgaggtcccatttgctaattcttcattttacagcacaagccattggtgttctgttcaaaaatctttccccctgaaccctatcttcgaggatcttccccactttctcctctataagtttcagtgtctctattattgtgctgaggggtaccgaagttcctattccgaagttcctattctctagaaagtataggaacttccctagggtttaaacccgcggtggagctctgatgtgggaacgcttcagtgttcaggaaccatatgatttatttaaaatatagaatcaaaagtaccaatttgcagttttgaaagatttattccagtgtaagcattagcaatgcaccaacatcaggtgatttctgaatccaacacgtcttatgtcctcatgatattaaaaaaaaaaaaaggccatccagaactgtgaacttgagttctaccttgttccctactgacattcagattttcttttttgcattctctttatcttacaggagacaggaggggagggctaactcattttactttggcttgtcccttgctggtccttgcccagaacgtaaagtagcttgcaagtcttcaaatctaaaaatcttagtaactcctacacgagtggcaatgccaaagagcagtgcaacaaagaggaagtaaatacgaccaaagagtattcttaaatacaccactggctcttgtttttgttttattgtgtgcctttgaactggaggggacccactgtctatgctcccacttagtccctcttctttgcactctggaggcttccaaccaaaatgacaatggcaattccgatgattgttacacactcctctaaaactgcatttttctggggtgcagtcataacccaaatgagataaacttccactgcaagctccttgatcacagaacttacttttggagcagggggtaccatgtctcaccattccagcatctgttgtttctgtcccacgatgttcatcaagcccaaagcaggtaaacccagagataatcgattgatggaatgaaacatgttcttgcaaatatggaagattggtgacattggtacactgcaaccttccacacagcttgtcctgatcagcacaagcattgaatgtgaggctttcttctgctctagtacaatgcccaaatcgaaaccgttgtttgttgatgtcatagcacttaatattagcattcttagcacttacaccaaagatttccatgcattgtatgttgcgatcagtgcagttacctttatagcagtaaccatcttctgagcatggtgtcccatcttgcagataagtgtcatctgggcaaatgtatttagtcccattacagtactctggaagatcacatatgttctggataggtctgcagagtgtcccagaaggactgtaagtgcaatttgcacagcataattctttatcacaaatgctaccaggtgttaacctgcaatcatttccacagcagggatctgaataacatgccttttgggagccacagtcacactgctcatcgttatctactttgaagtttccacaaaacttataagtcaatgatgtattataataaacatgacggtcatagaaaagacatggcatcagaccaggagtattaagtatgttgcttatctctgcaagggaacaattgctgaaagcatctgttaattgaggatgtctgaacataatgcaggtgttccttctctggcagacacagtacccctcatcatattttaagcctaaactccttccaacacgattggttattataggagataaaaataaaggatttcgatcatatttaccaatacaaattagggctaaggaagaacatatactcctctcagctggattaacctggttatcttgtggcccatacttattaagtaaaactcctgcatcaggcttaaatttattataaaagactgacacatagtaattataagccgaccctcctggaactgcaaactcaagtcgaaatggatcagaattggtgtacacagtcatgagaaagacatagtaccgcatatgaagattggtcagataggtgtccattaaactaatgacttgaaacaaatacccaacagtagatgaaagtttgtcacctgcagcagaattatatacagaattggttgcttgaaagtggccttttatagcagctggatgtgtagcgtagttcttactagatattctgggagctccatctgcatattccaatctggaggagggagaacctgtattatggctccagtgcttccatgcattcataggccctgtgtcatcagactcagatactatctgagaaacaaggtgttcaaagctctgtgaatcattgaggggtttgatttcataggtaaggtcatctaacttcatgacccctgacaggcccccataacaagtatccacagtgaccatggattgtgggatcccctccaggtagccaatatagtaacaatctacaggaaaaaaggggtaatccatctgtaaggctccttggtcatcttgagttgtcagcaacaagtgtctgggccaaatgagtgtctttctccgcaggtggatgatatgtctctggccccgaaaatgcaagctatatgagagcagtctttgtgcttgaagtcctttggtatggtagatctccttccgaggaataaccacctccgatgagatgtaacgccaagtaggatggccttgagaacaccagactggaaccaggaggagcagccagagtgcaaatagcaagaggaggaccctggggaccacaggtctttccactagcctcatgccccaggtcagagataacatcctgggtggagctaaatccctctgctgtggccactgcctggtctagaaaatactgacagaggactaaaaacctcctcaggctcccaacctaagtggttacccagacaactggagttaggtaacagtcactgggtgtggcaggaattgagtctgaatgtgttagctgaggttgaggttaaatattgtcaaaagggatgtctataaatgtgcctggacaagaaaagtcagaagcagcaaggagtgtctctgacaggctcaatcctttcttttctttttttgaagttcaaaatatcatttccacgtgaatgtatttggttcccagtgtgactctgggtctctttctaggagtcaatatttctttatatcttggctcatgtttctcacagttgttctaatttcttgttttgttttgtttgtttgtttgaacgttagtagtaaatactgtctatattagccttttagctataaatgattgtttttatttcttctaatcatattttgtttgagttttggttaaactatttacaaatgagttttttttttttccttttgggtgttgctcgaaagtttggagctttctgttaatattgtgttgttatttttccaatattattagacctgagaattctatctgggtacctgtgaactctagaatttttaaaaattccatctcttgggaacattacctctgaccccgtctgaggccgaagtggctgtccccctccaacctttagtatctttctttcctgactattgggatttcttcaagcaatcaggctgatgggttctcagcagtgagaccagtagactgccggtatgaacgtcgaagagactgccacacactccaggttcatcaacagtgctttcgcgtctcttacttttgtagaaggaaaagcagcctctgagttatctccaagaaatcattaatgaaagagttaaaagatgggtatcacccggagttcatgacaagccctggctcagacacgtgagcaaggtctacagccccaaagataggctgccctgcaacatgtatttataagatagaagaaaaaaatgggtggttggagggttgatcaacttacttcctctcaaacatatatatctcatctaagtgtgcaggggaaaactctgtaggactactgggattgttattatcattattattattattattattattattattattattattattattaacttaaggcattttattagatattttcttcatttagttttcaaatgttatccccggaacctcctatactctctccctgccctgctccccaacccacccactcctacatcctggccctggcattcccctatactgtggcagatgatcttcgtaagaccaagagcctttcctcccattgatggcctactaggctatcctcttttacatatgcaactagagtcacagctctggggaggtattgcttagttcatattgtttttcctcctatagggttgcagatccctttagctccttgggtactttctctagctcctccattgggggccctgtgttccatccaatagatgactgtgagcatccacttctgtatttgccaggtattggcatggatcttactgcaccttctgaactctctaagcagctttcctggtcacctccaggagcctcatgaataagtctctgcttcccccttgtggctatgagcattactgcacctgatacaccctgcagcttcctagggaagagggaggaagtggcttggcccctgtctggttaaggtaagaggagataaatcccttctcatgaattagggtgagaagggtcatgtgctctatcattggtgaccaacttggggacatgggcttatacagtcatcactctgaggctctgtgtaccaccagactgaactcccatatcctacatgcacataggacaacaccaagtagaaggaggttttaggactaaactgaaggacagagatggggtttctaaacaactagggagtgccagggccagcctctctaaccactataggacactatggagtctggttacaaagagagattactcaaggtccttagcactgattacagagcatatctcagatgccttctgctgaccagatgtatctttgcataatctgcctatccagattcagaaaattgatgccacatagccaagtggactttcaggaacagacgatttaaaaacaggcagagagatgtgagagaaaggagaaggagagagagaagggagagggagagaagagagagggagacggagaaggaaagagggagaaggagaaggagagaaggggcatggacagagggagggacagaaggagagaggagatagagagggggataaggaagaaaggagggagggagagagagagaaggctaagtctttccatacctgggtcccaatacctcttataacccaagcacatggtttcagatatcacaatgcggttgggatatagataactgtaaatacttgtgaaaataatggggctgagatctggggttttcatgatagtttcaaagtcactgtactgactaaaaccttccactggcccatctccagcttgttaatctgagggtatcaaatttcccactaagtgtgtttagaaagatctccacctttttgccctagtcttccagtgccccacctacgttctggtctcccacatctgatgtcttctcagtgattctggccctgcctgctccacagctacaaaccccttcctataatgagctctgtgctgagccatcatcctgaatcaatccaccttaagcagatgttttgcttatttttcctgtgtccatactacagaggaagggtaggcatgtagaagctgaggcatctcatctcactctaagcaccctcagtctctaaatgtgcccctttgtttccagcagttcagcctcaagcatcttttattcactcgtcttagagggacacatgtgctgtagtgttataagatgaaatttaaagcattagttattcccaacaagccaattaaacaagccaaaaacattcatcagtcattcccatggaacctctgaagcatcttcctgctctaaccttgagtttcctagggctgctgtgggatcacaggagctgtcctgtttaccagcctatcctgtcccacgggattcagttattagtgggtgcgagggggaccgcaaacctggaagaaaatgggattggaagagaaaagagaaacgaagaccaagtagatcttttcctatcaaggtcttcgtttattaggctgaggtgcctggtgtaaagcatgcatcgcggggaataggaaggggtcgagggggaattttacaaagaacaaagaagcgggcatctgctgacatgagggccgaagtcaggctccaggcagcgggagctccaccgcggtggcgccatttcattacctctttctccgcacccgacatagataaagctta

SEQ ID NO: 4 - DNA, 251 bp, synthetic construct
  source 1..251: mol_type = other DNA; note = synthetic
ccagcttcattagtaatcgttcatctgtggtaaaaaggcaggatttgaagcgatggaagatgggagtacggggcgttggaagacaaagtgccacacagcgcagccttcgtctagacccccgggctaactataacggtcctaaggtagcgaggggatgacagattctctgttcagtgcactcagggtctgcctccacgagaatcaccatgccctttctcaagactgtgttctgtgcagtgccctgtcagtgg

SEQ ID NO: 5 - DNA, 245 bp, synthetic construct
  source 1..245: mol_type = other DNA; note = synthetic
aggggtcgagggggaattttacaaagaacaaagaagcgggcatctgctgacatgagggccgaagtcaggctccaggcagcgggagctccaccgcggtggcgccatttcattacctctttctccgcacccgacatagataaagcttatcccccaccaagcaaatccccctacctggggccgagcttcccgtatgtgggaaaatgaatccctgaggtcgattgctgcatgcaatgaaattcaactag

SEQ ID NO: 6 - DNA, 21 bp, synthetic construct
  source 1..21: mol_type = other DNA; note = synthetic
caggtacagctgcagcagtca

SEQ ID NO: 7 - DNA, 21 bp, synthetic construct
  source 1..21: mol_type = other DNA; note = synthetic
ggagatggcacaggtgagtga

SEQ ID NO: 8 - DNA, 17 bp, synthetic construct
  source 1..17: mol_type = other DNA; note = synthetic
tccaggactggtgaagc

SEQ ID NO: 9 - DNA, 24 bp, synthetic construct
  source 1..24: mol_type = other DNA; note = synthetic
tagtcccagtgatgagaaagagat

SEQ ID NO: 10 - DNA, 24 bp, synthetic construct
  source 1..24: mol_type = other DNA; note = synthetic
gagaacacagaagtggatgagatc

SEQ ID NO: 11 - DNA, 17 bp, synthetic construct
  source 1..17: mol_type = other DNA; note = synthetic
tgagtccagtccaggga

SEQ ID NO: 12 - DNA, 28 bp, synthetic construct
  source 1..28: mol_type = other DNA; note = synthetic
aaaaattgagtgtgaatggataagagtg

SEQ ID NO: 13 - DNA, 21 bp, synthetic construct
  source 1..21: mol_type = other DNA; note = synthetic
aaccctggtcagaaactgcca

SEQ ID NO: 14 - DNA, 19 bp, synthetic construct
  source 1..19: mol_type = other DNA; note = synthetic
agagaaacagtggatacgt

SEQ ID NO: 15 - DNA, 22 bp, synthetic construct
  source 1..22: mol_type = other DNA; note = synthetic
aactacgcacagaagttccagg

SEQ ID NO: 16 - DNA, 18 bp, synthetic construct
  source 1..18: mol_type = other DNA; note = synthetic
gctcgtggatttgtccgc

SEQ ID NO: 17 - DNA, 16 bp, synthetic construct
  source 1..16: mol_type = other DNA; note = synthetic
cagagtcacgattacc

SEQ ID NO: 18 - DNA, 19 bp, synthetic construct
  source 1..19: mol_type = other DNA; note = synthetic
tgagcagcaccctcacgtt

SEQ ID NO: 19 - DNA, 23 bp, synthetic construct
  source 1..23: mol_type = other DNA; note = synthetic
gtggcctcacaggtatagctgtt

SEQ ID NO: 20 - DNA, 18 bp, synthetic construct
  source 1..18: mol_type = other DNA; note = synthetic
accaaggacgagtatgaa

SEQ ID NO: 21 - DNA, 33 bp, synthetic construct
  source 1..33: mol_type = other DNA; note = synthetic
gctagtagtggggcctacaggccttttgatatc

SEQ ID NO: 22 - DNA, 48 bp, synthetic construct
  source 1..48: mol_type = other DNA; note = synthetic
gcaaaagcccaggggagtgggagctactacacctatgcttttgatatc

SEQ ID NO: 23 - DNA, 42 bp, synthetic construct
  source 1..42: mol_type = other DNA; note = synthetic
gcgagagagggtatagtgggaactactgaggactttgattac

SEQ ID NO: 24 - DNA, 33 bp, synthetic construct
  source 1..33: mol_type = other DNA; note = synthetic
gcgagagggacagtgggagccctctttgactac

SEQ ID NO: 25 - DNA, 36 bp, synthetic construct
  source 1..36: mol_type = other DNA; note = synthetic
gcgaaacctagtgggagctactcctggttcgacccc

SEQ ID NO: 26 - DNA, 45 bp, synthetic construct
  source 1..45: mol_type = other DNA; note = synthetic
gcgagaggaggagggtataactggaactcgaatgcttttgatatc

SEQ ID NO: 27 - DNA, 33 bp, synthetic construct
  source 1..33: mol_type = other DNA; note = synthetic
gcgagaggatataactggaactactttgactac

SEQ ID NO: 28 - DNA, 39 bp, synthetic construct
  source 1..39: mol_type = other DNA; note = synthetic
gcgaaagagtataactggaaccactggtactttgactac

SEQ ID NO: 29 - DNA, 33 bp, synthetic construct
  source 1..33: mol_type = other DNA; note = synthetic
gcgagagagataactggaaccccctttgactac

SEQ ID NO: 30 - DNA, 39 bp, synthetic construct
  source 1..39: mol_type = other DNA; note = synthetic
gcgaggggatataactggaacttttctttttttgactac

SEQ ID NO: 31 - DNA, 36 bp, synthetic construct
  source 1..36: mol_type = other DNA; note = synthetic
gcgagaggtaactggaactctctgggctttgactac

SEQ ID NO: 32 - DNA, 39 bp, synthetic construct
  source 1..39: mol_type = other DNA; note = synthetic
gcgaaaagggctactatggttcggggagctcttgactac

SEQ ID NO: 33 - DNA, 60 bp, synthetic construct
  source 1..60: mol_type = other DNA; note = synthetic
gcgagagatattactatggttcggggagttattataacgaaggtctacggtatggacgtc

SEQ ID NO: 34 - DNA, 27 bp, synthetic construct
  source 1..27: mol_type = other DNA; note = synthetic
gcgagagagtatagcagctttgactac

SEQ ID NO: 35 - DNA, 33 bp, synthetic construct
  source 1..33: mol_type = other DNA; note = synthetic
gcgagagagagtatagcagctcgttgtgactac

SEQ ID NO: 36 - DNA, 42 bp, synthetic construct
  source 1..42: mol_type = other DNA; note = synthetic
gcaagagaggataggagctcgcccctcgggtactttgactac

SEQ ID NO: 37 - DNA, 24 bp, synthetic construct
  source 1..24: mol_type = other DNA; note = synthetic
gcgagagatcttggggaaggctac

SEQ ID NO: 38 - DNA, 30 bp, synthetic construct
  source 1..30: mol_type = other DNA; note = synthetic
accacccataactggggagggtttgactac

SEQ ID NO: 39 - DNA, 18 bp, synthetic construct
  source 1..18: mol_type = other DNA; note = synthetic
gcgagagataggggaccg

SEQ ID NO: 40 - DNA, 30 bp, synthetic construct
  source 1..30: mol_type = other DNA; note = synthetic
caacagagttatagtacccctccggagacg

SEQ ID NO: 41 - DNA, 27 bp, synthetic construct
  source 1..27: mol_type = other DNA; note = synthetic
caacagcttaatagttaccctcggacg

SEQ ID NO: 42 - DNA, 26 bp, synthetic construct
  source 1..26: mol_type = other DNA; note = synthetic
caacagcttaatagttaccattcact

SEQ ID NO: 43 - DNA, 27 bp, synthetic construct
  source 1..27: mol_type = other DNA; note = synthetic
caacattttaatagttacccgctcact

SEQ ID NO: 44 - DNA, 27 bp, synthetic construct
  source 1..27: mol_type = other DNA; note = synthetic
cagcagtataataactggcctctcact

SEQ ID NO: 45 - DNA, 27 bp, synthetic construct
  source 1..27: mol_type = other DNA; note = synthetic
ctacagcataatagttacccgtggacg

SEQ ID NO: 46 - DNA, 27 bp, synthetic construct
  source 1..27: mol_type = other DNA; note = synthetic
ctacagcataatagttaccctcggacg

SEQ ID NO: 47 - DNA, 27 bp, synthetic construct
  source 1..27: mol_type = other DNA; note = synthetic
cagcagtatggtagctcacctcggacg

SEQ ID NO: 48 - DNA, 27 bp, synthetic construct
  source 1..27: mol_type = other DNA; note = synthetic
atgcaaggtacacactggccgtggacg

SEQ ID NO: 49 - DNA, 27 bp, synthetic construct
  source 1..27: mol_type = other DNA; note = synthetic
atgcaaggttcacactggccgtacact

SEQ ID NO: 50 - DNA, 27 bp, synthetic construct
  source 1..27: mol_type = other DNA; note = synthetic
atgcaaggtacacactggccgctcact

SEQ ID NO: 51 - DNA, 27 bp, synthetic construct
  source 1..27: mol_type = other DNA; note = synthetic
caacagtatgataatctccctcccact

SEQ ID NO: 52 - DNA, 27 bp, synthetic construct
  source 1..27: mol_type = other DNA; note = synthetic
caacagtatgataatctcccattcact

SEQ ID NO: 53 - DNA, 27 bp, synthetic construct
  source 1..27: mol_type = other DNA; note = synthetic
caacagtatgataatctccccgtcact

SEQ ID NO: 54 - DNA, 27 bp, synthetic construct
  source 1..27: mol_type = other DNA; note = synthetic
caacagtatgataatctcccgatcacc

SEQ ID NO: 55 - DNA, 24 bp, synthetic construct
  source 1..24: mol_type = other DNA; note = synthetic
caacggatttacaatgccgacacc

SEQ ID NO: 56 - DNA, 30 bp, synthetic construct
  source 1..30: mol_type = other DNA; note = synthetic
caacagagttacagtacccccatgtacact

SEQ ID NO: 57 - DNA, 27 bp, synthetic construct
  source 1..27: mol_type = other DNA; note = synthetic
caacagagttacagtacccctctcact

SEQ ID NO: 58 - DNA, 27 bp, synthetic construct
  source 1..27: mol_type = other DNA; note = synthetic
caacagagttacagtactcctcccact

SEQ ID NO: 59 - DNA, 219 bp, synthetic construct
  source 1..219: mol_type = other DNA; note = synthetic
actttcagaatgttcttgaacagtctctgagaaacacggaagacggccgcataacttcgtatagtatacattatacgaagttattctagacccccgggctcgataactataacggtcctaaggtagcgactcgagataacttcgtataatgtatgctatacgaagttatccatggtaagcttacgtggcatacagtgtcagattttctgtttatcaagc

SEQ ID NO: 60 - DNA, 21 bp, synthetic construct
  source 1..21: mol_type = other DNA; note = synthetic
agctgaatggaaacaaggcaa

SEQ ID NO: 61 - DNA, 19 bp, synthetic construct
  source 1..19: mol_type = other DNA; note = synthetic
ggagacaatgccccagtga

SEQ ID NO: 62 - DNA, 21 bp, synthetic construct
  source 1..21: mol_type = other DNA; note = synthetic
tcccatagggctaggatttcc

SEQ ID NO: 63 - DNA, 19 bp, synthetic construct
  source 1..19: mol_type = other DNA; note = synthetic
tcccctcacactgttcccc

SEQ ID NO: 64 - DNA, 19 bp, synthetic construct
  source 1..19: mol_type = other DNA; note = synthetic
ggtggagaggctattcggc

SEQ ID NO: 65 - DNA, 17 bp, synthetic construct
  source 1..17: mol_type = other DNA; note = synthetic
gaacacggcggcatcag

SEQ ID NO: 66 - DNA, 21 bp, synthetic construct
  source 1..21: mol_type = other DNA; note = synthetic
tcaacctttcccagcctgtct

SEQ ID NO: 67 - DNA, 24 bp, synthetic construct
  source 1..24: mol_type = other DNA; note = synthetic
ccccagagagagaaaacagatttt

SEQ ID NO: 68 - DNA, 20 bp, synthetic construct
  source 1..20: mol_type = other DNA; note = synthetic
ccctggtgaagcatgtttgc

SEQ ID NO: 69 - DNA, 20 bp, synthetic construct
  source 1..20: mol_type = other DNA; note = synthetic
tgtggcctgtctgccttacg

SEQ ID NO: 70 - DNA, 21 bp, synthetic construct
  source 1..21: mol_type = other DNA; note = synthetic
cacacctagaccccggaagtc

SEQ ID NO: 71 - DNA, 21 bp, synthetic construct
  source 1..21: mol_type = other DNA; note = synthetic
tcgctttgccagttgattctc

SEQ ID NO: 72 - DNA, 17 bp, synthetic construct
  source 1..17: mol_type = other DNA; note = synthetic
tgcggccgatcttagcc

SEQ ID NO: 73 - DNA, 18 bp, synthetic construct
  source 1..18: mol_type = other DNA; note = synthetic
ttgaccgattccttgcgg

SEQ ID NO: 74 - DNA, 20 bp, synthetic construct
  source 1..20: mol_type = other DNA; note = synthetic
gcaaacaaaaaccactggcc

SEQ ID NO: 75 - DNA, 19 bp, synthetic construct
  source 1..19: mol_type = other DNA; note = synthetic
ggccacattccatgggttc

SEQ ID NO: 76 - DNA, 22 bp, synthetic construct
  source 1..22: mol_type = other DNA; note = synthetic
ccatgactgggcctctgtagac

SEQ ID NO: 77 - DNA, 25 bp, synthetic construct
  source 1..25: mol_type = other DNA; note = synthetic
caagtcagggtgctaatgctgtatc

SEQ ID NO: 78 - DNA, 19 bp, synthetic construct
  source 1..19: mol_type = other DNA; note = synthetic
cacagcttgtgcagcctcc

SEQ ID NO: 79 - DNA, 22 bp, synthetic construct
  source 1..22: mol_type = other DNA; note = synthetic
gggcactggatacgatgtatgg

SEQ ID NO: 80 - DNA, 21 bp, synthetic construct
  source 1..21: mol_type = other DNA; note = synthetic
tcataggtaggtctcagtttg

SEQ ID NO: 81 - DNA, 21 bp, synthetic construct
  source 1..21: mol_type = other DNA; note = synthetic
tgatctgcgctgtttcatcct

SEQ ID NO: 82 - DNA, 31 bp, synthetic construct
  source 1..31: mol_type = other DNA; note = synthetic
tgacatgaaccatctgtttctctctcgacaa

SEQ ID NO: 83 - DNA, 29 bp, synthetic construct
  source 1..29: mol_type = other DNA; note = synthetic
agagacgctccgaggtcaaggtgctctag

SEQ ID NO: 84 - DNA, 23 bp, synthetic construct
  source 1..23: mol_type = other DNA; note = synthetic
tgggcacaacagacaatcggctg

SEQ ID NO: 85 - DNA, 16 bp, synthetic construct
  source 1..16: mol_type = other DNA; note = synthetic
accctctgctgtccct

SEQ ID NO: 86 - DNA, 26 bp, synthetic construct
  source 1..26: mol_type = other DNA; note = synthetic
ccaagcaggaggtgctcagttcccaa

SEQ ID NO: 87 - DNA, 24 bp, synthetic construct
  source 1..24: mol_type = other DNA; note = synthetic
tccacactgtcggctgggagctca

SEQ ID NO: 88 - DNA, 21 bp, synthetic construct
  source 1..21: mol_type = other DNA; note = synthetic
acgagcgggttcggcccattc

SEQ ID NO: 89 - DNA, 37 bp, synthetic construct
  source 1..37: mol_type = other DNA; note = synthetic
ctgttcctctaaaactggactccacagtaaatggaaa

SEQ ID NO: 90 - DNA, 27 bp, synthetic construct
  source 1..27: mol_type = other DNA; note = synthetic
tgccgcttatacaacactgccatctgc

SEQ ID NO: 91 - DNA, 37 bp, synthetic construct
  source 1..37: mol_type = other DNA; note = synthetic
agaagaagcctgtactacagcatccgttttacagtca

SEQ ID NO: 92 - DNA, 21 bp, synthetic construct
  source 1..21: mol_type = other DNA; note = synthetic
gggctacttgaggaccttgct

SEQ ID NO: 93 - DNA, 23 bp, synthetic construct
  source 1..23: mol_type = other DNA; note = synthetic
gacagcccttacagagtttggaa

SEQ ID NO: 94 - DNA, 23 bp, synthetic construct
  source 1..23: mol_type = other DNA; note = synthetic
aagaccaggagctctgcctaagt

SEQ ID NO: 95 - DNA, 22 bp, synthetic construct
  source 1..22: mol_type = other DNA; note = synthetic
cccatcacgaactgaagttgag

SEQ ID NO: 96 - DNA, 20 bp, synthetic construct
  source 1..20: mol_type = other DNA; note = synthetic
cagggcctccatcccaggca

SEQ ID NO: 97 - DNA, 28 bp, synthetic construct
  source 1..28: mol_type = other DNA; note = synthetic
ccccagtgtgtgaatcactctaccctcc

SEQ ID NO: 98 - DNA, 20 bp, synthetic construct
  source 1..20: mol_type = other DNA; note = synthetic
cctctcctcctcaccctcct

SEQ ID NO: 99 - DNA, 20 bp, synthetic construct
  source 1..20: mol_type = other DNA; note = synthetic
  misc_difference 4: note = variation - r=a or g
  misc_difference 9: note = variation - s=c or g
  misc_difference 11: note = variation - y=c or t
  misc_difference 12: note = variation - y=c or t
  misc_difference 13: note = variation - y=c or t
atgrccdgstyyyctctcct

SEQ ID NO: 100 - DNA, 18 bp, synthetic construct
  source 1..18: mol_type = other DNA; note = synthetic
ctcctcactcagggcaca

SEQ ID NO: 101 - DNA, 20 bp, synthetic construct
  source 1..20: mol_type = other DNA; note = synthetic
  misc_difference 18: note = variation - s=c or g
atggcctgggctctgctsct

SEQ ID NO: 102 - DNA, 19 bp, synthetic construct
  source 1..19: mol_type = other DNA; note = synthetic
  misc_difference 11: note = variation - y=c or t
  misc_difference 13: note = variation - s=c or g
atggcctggaycsctctcc

SEQ ID NO: 103 - DNA, 23 bp, synthetic construct
  source 1..23: mol_type = other DNA; note = synthetic
  misc_difference 11: note = variation - y=c or t
  misc_difference 15: note = variation - r=a or g
  misc_difference 16: note = variation - y=c or t
  misc_difference 18: note = variation - y=c or t
  misc_difference 20: note = variation - m=a or c
  misc_difference 21: note = variation - y=c or t
tcaccatggcytggrycycmytc

SEQ ID NO: 104 - DNA, 22 bp, synthetic construct
  source 1..22: mol_type = other DNA; note = synthetic
tcaccatggcctgggtctcctt

SEQ ID NO: 105 - DNA, 22 bp, synthetic construct
  source 1..22: mol_type = other DNA; note = synthetic
  misc_difference 16: note = variation - m=a or c
  misc_difference 19: note = variation - y=c or t
tcaccatggcctggamtcytct

SEQ ID NO: 106 - DNA, 26 bp, synthetic construct
  source 1..26: mol_type = other DNA; note = synthetic
tcaccatggcctgggctccactactt

SEQ ID NO: 107 - DNA, 20 bp, synthetic construct
  source 1..20: mol_type = other DNA; note = synthetic
tcaccatggcctggactcct

SEQ ID NO: 108 - DNA, 23 bp, synthetic construct
  source 1..23: mol_type = other DNA; note = synthetic
tcaccatggcctggatgatgctt

SEQ ID NO: 109 - DNA, 22 bp, synthetic construct
  source 1..22: mol_type = other DNA; note = synthetic
taaatatggcctgggctcctct

SEQ ID NO: 110 - DNA, 22 bp, synthetic construct
  source 1..22: mol_type = other DNA; note = synthetic
tcaccatgccctgggctctgct

SEQ ID NO: 111 - DNA, 22 bp, synthetic construct
  source 1..22: mol_type = other DNA; note = synthetic
tcaccatggccctgactcctct

SEQ ID NO: 112 - DNA, 30 bp, synthetic construct
  source 1..30: mol_type = other DNA; note = synthetic
cccaagcttactggatggtgggaagatgga

SEQ ID NO: 113 - DNA, 16 bp, synthetic construct
  source 1..16: mol_type = other DNA; note = synthetic
gtaaaacgacggccag

SEQ ID NO: 114 - DNA, 17 bp, synthetic construct
  source 1..17: mol_type = other DNA; note = synthetic
caggaaacagctatgac

SEQ ID NO: 115 - DNA, 440 bp, synthetic construct
  source 1..440: mol_type = other DNA; note = synthetic
gggcctgggctctgctgctcctcaccctcctcactcagggcacagggtcctgggcccagtctgccctgactcagcctccctccgcgtccgggtctcctggacagtcagtcaccatctcctgcactggaaccagcagtgacgttggtggttataactatgtctcctggtaccaacagcacccaggcaaagcccccaaactcatgatttatgaggtcagtaagcggccctcaggggtccctgatcgcttctctggctccaagtctggcaacacggcctccctgaccgtctctgggctccaggctgaggatgaggctgattattactgcagctcatatgcaggcagcaacaatttcgtcttcggaactgggaccaaggtcaccgtcctaggggctgatgctgcaccaactgtatccatcttcccaccatccagtaagcttggg

SEQ ID NO: 116 - DNA, 441 bp, synthetic construct
  source 1..441: mol_type = other DNA; note = synthetic
atggcctgggctctgctgctcctcaccctcctcactcagggcacagggtcctgggcccagtctgccctgactcagcctccctccgcgtccgggtctcctggacagtcagtcaccatctcctgcactggaaccagcagtgacgttggtggttataactatgtctcctggtaccaacagcacccaggcaaagcccccaaactcatgatttatgaggtcactaagcggccctcaggggtccctgatcgcttctctggctccaagtctggcaacacggcctccctgaccgtctctgggctccaggctgaggatgaggctgattattactgcagctcatatgcaggcagcaacaattatgtcttcggaactgggaccaaggtcaccgtcctaggggctgatgctgcaccaactgtatccatcttcccaccatccagtaagcttggg

SEQ ID NO: 117 - DNA, 441 bp, synthetic construct
  source 1..441: mol_type = other DNA; note = synthetic
atggcctgggctctgctgctcctcaccctcctcactcagggcacagggtcctgggcccagtctgccctgactcagcctccctccgcgtccgggtctcctggacagtcagtcaccatctcctgcactggaaccagcagtgacgttggtggttataactatgtctcctggtaccaacagcacccaggcaaagcccccaaactcatgatttatgaggtcagtaagcggccctcaggggtccctgatcgcttctctggctccaagtctggcaacacggcctccctgaccgtctctgggctccaggctgaggatgaggctgattattactgcagctcatatgcaggcagcaacaattatgtcttcggaactgggaccaaggtcaccgtcctaggggctgatgctgcaccaactgtatccatcttcccaccatccagtaagcttggg

SEQ ID NO: 118 - DNA, 438 bp, synthetic construct
  source 1..438: mol_type = other DNA; note = synthetic
atggcctgggctctgctcctcaccctcctcactcagggcacagggtcctgggcccagtctgccctgactcagcctccctccgcgtccgggtctcctggacagtcagtcaccatctcctgcactggaaccagcagtgacgttggtggttataactatgtctcctggtaccaacagcacccaggcaaagcccccaaactcatgatttatgaggtcagtaagcggccctcaggggtccctgatcgcttctctggctccaagtctggcaacacggcctccctgaccgtctctgggctccaggctgaggatgaggctgattattactgcagctcatatgcaggcagcaacaattatgtcttcggaactgggaccaaggtcaccgtcctaggggctgatgctgcaccaactgtatccatcttcccaccatccagtaagcttggg

SEQ ID NO: 119 - DNA, 438 bp, synthetic construct
  source 1..438: mol_type = other DNA; note = synthetic
atggcctgggctctgctgctcctcaccctcctcactcagggcacagggtcctgggcccagtctgccctgactcagcctccctccgcgtccgggtctcctggacagtcagtcaccatctcctgcactggaaccagcagtgacgttggtggttataactatgtctcctggtaccaacagcacccaggcaaagcccccaaactcatgatttatgaggtcagtaagcggccctcaggggtccctgatcgcttctctggctccaagtctggcaacacggcctccctgaccgtctctgggctccaggctgaggatgaggctgattattactgcagctcatatgcaggcagcaacaatgtcttcggaactgggaccaaggtcaccgtcctaggggctgatgctgcaccaactgtatccatcttcccaccatccagtaagcttggg

SEQ ID NO: 120 - DNA, 441 bp, synthetic construct
  source 1..441: mol_type = other DNA; note = synthetic
atggcctgggctctgctcctcctcaccctcctcactcagggcacagggtcctgggcccagtctgccctgactcagcctccctccgcgtccgggtctcctggacagtcagtcaccatctcctgcactggaaccagcagtgacgttggtggttataactatgtctcctggtaccaacagcacccaggcaaagcccccaaactcatgatttatgaggtcagtaagcggccctcaggggtccctgatcgcttctctggctccaagtctggcaacacggcctccctgaccgtctctgggctccaggctgaggatgaggctgattattactgcagctcatatgcaggcagcaacaattatgtcttcggaactgggaccaaggtcaccgtcctaggggctgatgctgcaccaactgtatccatcttcccaccatccagtaagcttggg

SEQ ID NO: 121 - DNA, 442 bp, synthetic construct
  source 1..442: mol_type = other DNA; note = synthetic
atggcctgggctctgctgctcctcaccctcctcactcagggcacagggtcctgggcccagtctgccctgactcagcctccctccgcgtccgggtctcctggacagtcagtcaccatctcctgcactggaaccagcagtgacgttggtggttataactatgtctcctggtaccaacagcacccaggcaaagcccccaaactcatgatttatgaggtcagtaagcggccctcaggggtccctgatcgcttctctggctccaagtctggcaacacggcctccctgaccgtctctgggctccaggctgaggatgaggctgattattactgcagctcatatgcaggcagcaacaatttatgtcttcggaactgggaccaaggtcaccgtcctaggggctgatgctgcaccaactgtatccatcttcccaccatccagtaagcttggg

SEQ ID NO: 122 - DNA, 428 bp, synthetic construct
  source 1..428: mol_type = other DNA; note = synthetic
ccttcattttctccacaggtctctgtgctctgcctgtgctgactcagcccccgtctgcatctgccttgctgggagcctcgatcaagctcacctgcaccctaagcagtgagcacagcacctacaccatcgaatggtatcaacagagaccagggaggtccccccagtatataatgaaggttaagagtgatggcagccacagcaagggggacgggatccccgatcgcttcatgggctccagttctggggctgaccgctacctcaccttctccaacctccagtctgacgatgaggctgagtatcactgtggagagagccacacgattgatggccaagtcggttgtgtcttcggaactgggaccaaggtcaccgtcctaggggctgatgctgcaccaactgtatccatcttcccaccatccagtaagcttggg

SEQ ID NO: 123 - DNA, 441 bp, synthetic construct
  source 1..441: mol_type = other DNA; note = synthetic
atgacctgctcccctctcctcctcacccttctcattcactgcacagggtcctgggcccagtctgtgttgacgcagccgccctcagtgtctgcggccccaggacagaaggtcaccatctcctgctctggaagcagctccaacattgggaataattatgtatcctggtaccagcagctcccaggaacagcccccaaactcctcatttatgacaataataagcgaccctcagggattcctgaccgattctctggctccaagtctggcacgtcagccaccctgggcatcaccggactccagactggggacgaggccgattattactgcggaacatgggatagcagcctgagtgcttatgtcttcggaactgggaccaaggtcaccgtcctaggggctgatgctgcaccaactgtatccatcttcccaccatccagtgagcagtta

SEQ ID NO: 124 - DNA, 441 bp, synthetic construct
  source 1..441: mol_type = other DNA; note = synthetic
atgacctgctcccctctcctcctcacccttctcattcactgcacagggtcctgggcccagtctgtgttgacgcagccgccctcagtgtctgcggccccaggacagaaggtcaccatctcctgctctggaagcagctccaacattgggaataattatgtatcctggtaccagcagctcccaggaacagcccccaaactcctcatttatgacaataataagcgaccctcagggattcctgaccgattctctggctccaagtctggcacgtcagccaccctgggcatcaccggactccagactggggacgaggccgattattactgcggaacatgggatagcagcctgagtgcggctttttttggaactgggaccaaggtcaccgtcctaggggctgatgctgcaccaactgtatccatcttcccaccatccagtgagcagtta

SEQ ID NO: 125 - DNA, 345 bp, synthetic construct
  source 1..345: mol_type = other DNA; note = synthetic
cccgggcagagggtcaccatctcttgttctggaagcagctccaacatcggaagtaatactgtaaactggtaccagcagctcccaggaacggcccccaaactcctcatctatagtaataatcagcggccctcaggggtccctgaccgattctctggctccaagtctggcacctcagcctccctggccatcagtgggctccagtctgaggatgaggctgattattactgtgcagcatgggatgacagcctgaatggttatgtcttcggaactgggaccaaggtcaccgtcctaggggctgatgctgcaccaactgtatccatcttcccaccatccagtgagcagtta

SEQ ID NO: 126 - DNA, 432 bp, synthetic construct
  source 1..432: mol_type = other DNA; note = synthetic
atggcctggacccctctcctgctccccctcctcactttctgcacagtctctgaggcctcctatgagctgacacagccaccctcggtgtcagtgtccccaggacaaacggccaggatcacctgctctggagatgcattgccaaaaaaatatgcttattggtaccagcagaagtcaggccaggcccctgtgctggtcatctatgaggacagcaaacgaccctccgggatccctgagagattctctggctccagctcagggacaatggccaccttgactatcagtggggcccaggtggaggatgaagctgactactactgttactcaacagactacagtggtaatcatgtcttcggaactgggaccaaggtcaccgtcctaggggctgatgctgcaccaactgtatccatcttcccaccatccagtgagcagtta

SEQ ID NO: 127 - DNA, 426 bp, synthetic construct
  source 1..426: mol_type = other DNA; note = synthetic
atggcctggactcctctctttctgttcctcctcacttgctgcccagggtccaattcccaggctgtggtgactcaggagccctcactgactgtgtccccaggagggacagtcactctcacctgtggctccagcactggagctgtcaccagtggtcattatccctactggttccagcagaagcctggccaagcccccaggacactgatttatgatacaagcaacaaacactcctggacacctgcccggttctcaggctccctccttgggggcaaagctgccctgaccctttcgggtgcgcagcctgaggatgaggctgagtattactgcttgctctcctatagtggtgcttatgtcttcggaactgggaccaaggtcaccgtcctaggggctgatgctgcaccaactgtatccatcttcccaccatcc

SEQ ID NO: 128 - DNA, 331 bp, synthetic construct
  source 1..331: mol_type = other DNA; note = synthetic
agtggtcctgggacagacggccaggattacctgtgggggaaacaacattggaagtaaaaatgtgcactggtaccagcagaagccaggccaggcccctgtgctggtcatctatagggataacaaccggccctctgggatccctgagcgattctctggctccaactcggggaacacggccaccctgaccatcagcagagcccaagccggggatgaggctgactattactgtcaggtgtgggacagcagcacttatgtcttcggaactgggaccaaggtcaccgtcctaggggctgatgctgcaccaactgtatccatcttcccaccatccagt

SEQ ID NO: 129 - DNA, 417 bp, synthetic construct
  source 1..417: mol_type = other DNA; note = synthetic
actcctctcctcctcctgttcctctctcactgcacaggttccctctcgcaggctgtgctgactcagccgtcttccctctctgcatctcctggagcatcagccagtctcacctgcaccttgcgcagtggcatcaatgttggtacctacaggatatactggtaccagcagaagccagggagtcctccccagtatctcctgaggtacaaatcagactcagataagcagcagggctctggagtccccagccgcttctctggatccaaagatgcttcggccaatgcagggattttactcatctctgggctccagtctgaggatgaggctgactattactgtatgatttggcacagcagcgcttatgtcttcggaactgggaccaaggtcaccgtcctaggggctgatgctgcaccaactgta

SEQ ID NO: 130 - DNA, 393 bp, synthetic construct
  source 1..393: mol_type = other DNA; note = synthetic
tttctgttcctcctcacttgctgcccagggtccaattctcagactgtggtgactcaggagccctcactgactgtgtccccaggagggacagtcactctcacctgtgcttccagcactggagcagtcaccagtggttactatccaaactggttccagcagaaacctggacaagcacccagggcactgatttatagtacaagcaacaaacgctcctggacccctgcccggttctcaggctccctccttgggggcaaagctgccctgacactgtcaggtgtgcagcctgaggacgaggctgagtattactgcctgctctactatggtggtgcttatgtcttcggaactgggaccaaggtcaccgtcctaggggctgatgctgcaccaactgtatcc

SEQ ID NO: 131 - DNA, 417 bp, synthetic construct
  source 1..417: mol_type = other DNA; note = synthetic
atggcctgggctctgctgctcctcactctcctcactcaggacacagggtcctgggcccagtctgccctgactcagcctgcctccgtgtctgggtctcctggacagtcgatcaccatctcctgcactggaaccagcagtgatgttgggagttataaccttgtctcctggtaccaacagcacccaggcaaagcccccaaactcatgatttatgagggcagtaagcggccctcaggggtttctaatcgcttctctggctccaagtctggcaacacggcctccctgacaatctctgggctccaggctgaggacgaggctgattattactgctgctcatatgcaggtagtagcacttatgtcttcggaactgggaccaaggtcaccgtcctaggggctgatgctgcaccaactgtatccatc

SEQ ID NO: 132 - DNA, 348 bp, synthetic construct
  source 1..348: mol_type = other DNA; note = synthetic
cagtctgccctgactcagcctgcctccgtgtctgggtctcctggacagtcgatcaccatctcctgcactggaaccagcagtgacgttggtggttataactatgtctcctggtaccaacagcacccaggcaaagcccccaaactcatgatttatgaggtcagtaatcggccctcaggggtttctaatcgcttctctggctccaagtctggcaacacggcctccctgaccatctctgggctccaggctgaggacgaggctgattattactgcagctcatatacaagcagcagcacttatgtcttcggaactgggaccaaggtcaccggcctgggggctgatgctgcacca

SEQ ID NO: 133 - DNA, 20 bp, synthetic construct
  source 1..20: mol_type = other DNA; note = synthetic
aacaaccgagctccaggtgt

SEQ ID NO: 134 - DNA, 19 bp, synthetic construct
  source 1..19: mol_type = other DNA; note = synthetic
agggcagccttgtctccaa

SEQ ID NO: 135 - DNA, 20 bp, synthetic construct
  source 1..20: mol_type = other DNA; note = synthetic
cctgccagattctcaggctc

SEQ ID NO: 136 - DNA, 20 bp, synthetic construct
  source 1..20: mol_type = other DNA; note = synthetic
catcacaggggcacagactg

SEQ ID NO: 137 - DNA, 19 bp, synthetic construct
  source 1..19: mol_type = other DNA; note = synthetic
gatttgctgagggcagggt

SEQ ID NO: 138 - DNA, 21 bp, synthetic construct
  source 1..21: mol_type = other DNA; note = synthetic
ccccaagtctgatccttcctt

SEQ ID NO: 139 - DNA, 20 bp, synthetic construct
  source 1..20: mol_type = other DNA; note = synthetic
gctgaccaacgatcgcctaa

SEQ ID NO: 140 - DNA, 19 bp, synthetic construct
  source 1..19: mol_type = other DNA; note = synthetic
taagcgccacactgcacct

SEQ ID NO: 141 - DNA, 24 bp, synthetic construct
  source 1..24: mol_type = other DNA; note = synthetic
cctgccagattctcaggctccctg

SEQ ID NO: 142 - DNA, 23 bp, synthetic construct
  source 1..23: mol_type = other DNA; note = synthetic
ctgattggagacaaggctgccct

SEQ ID NO: 143 - DNA, 30 bp, synthetic construct
  source 1..30: mol_type = other DNA; note = synthetic
ccttcatactcttgcatcctcccttctcca

SEQ ID NO: 144 - DNA, 35 bp, synthetic construct
  source 1..35: mol_type = other DNA; note = synthetic
ttccttctcttctgtgactcaattatttgtggaca

SEQ ID NO: 145 - DNA, 159 bp, synthetic construct
  source 1..159: mol_type = other DNA; note = synthetic
tctggcacctcagcctccctggccatcactgggctccaggctgaggatgaggctgattattactgccagtcctatgacagcagcctgagtggttctgtgttcggaggaggcacccggctgaccgccctcggggctgatgctgcaccaactgtatccatc

SEQ ID NO: 146 - DNA, 159 bp, synthetic construct
  source 1..159: mol_type = other DNA; note = synthetic
tctggcacctcagcctccctggccatcactgggctccaggctgaggatgaggctgattattactgccagtcctatgacagcagcctgagtggttatgtcttcggaactgggaccaaggtcaccgtcctaggggctgatgctgcaccaactgtatccatc

SEQ ID NO: 147 - DNA, 159 bp, synthetic construct
  source 1..159: mol_type = other DNA; note = synthetic
tctggcacctcagcctccctggccatcagtgggctccagtctgaggatgaggctgattattactgtgcagcatgggatgacagcctgaatggtgctgtgttcggaggaggcacccagctgaccgccctcggggctgatgctgcaccaactgtatccatc

SEQ ID NO: 148 - DNA, 159 bp, synthetic construct
  source 1..159: mol_type = other DNA; note = synthetic
tctggcacctcagcctccctggccatcagtgggctccggtccgaggatgaggctgattattactgtgcagcatgggatgacagcctgagtggtcgggtgttcggcggagggaccaagctgaccgtcctaggggctgatgctgcaccaactgtatccatc

SEQ ID NO: 149 - DNA, 153 bp, synthetic construct
  source 1..153: mol_type = other DNA; note = synthetic
tcggggaacacggccaccctgaccatcagcagagcccaagccggggatgaggctgactattactgtcaggtgtgggacagcagcactgctgtgttcggaggaggcacccagctgaccgccctcggggctgatgctgcaccaactgtatccatc

SEQ ID NO: 150 - DNA, 156 bp, synthetic construct
  source 1..156: mol_type = other DNA; note = synthetic
tcagggacaatggccaccttgactatcagtggggcccaggtggaggatgaagctgactactactgttactcaacagacagcagtggtaatgctgtgttcggaggaggcacccagctgaccgccctcggggctgatgctgcaccaactgtatccatc

SEQ ID NO: 151 - DNA, 159 bp, synthetic construct
  source 1..159: mol_type = other DNA; note = synthetic
tcagggacaatggccaccttgactatcagtggggcccaggtggaggatgaagctgactactactgttactcaacagacagcagtggtaatcatagggtgttcggcggagggaccaagctgaccgtcctaggggctgatgctgcaccaactgtatccatc

SEQ ID NO: 152 - DNA, 159 bp, synthetic construct; identical to SEQ ID NO: 146
  source 1..159: mol_type = other DNA; note = synthetic

SEQ ID NO: 153 - DNA, 159 bp, synthetic construct
  source 1..159: mol_type = other DNA; note = synthetic
gatgcttcggccaatgcagggattttactcatctctgggctccagtctgaggatgaggctgactattactgtatgatttggcacagcagcgctgtggtattcggcggagggaccaagctgaccgtcctaggggctgatgctgcaccaactgtatccatc

SEQ ID NO: 154 - DNA, 153 bp, synthetic construct
  source 1..153: mol_type = other DNA; note = synthetic
cttgggggcaaagctgccctgacactgtcaggtgtgcagcctgaggacgaggctgagtattactgcctgctctactatggtggtgctcgggtgttcggcggagggaccaagctgaccgtcctaggggctgatgctgcaccaactgtatccatc

SEQ ID NO: 155 - DNA, 153 bp, synthetic construct
  source 1..153: mol_type = other DNA; note = synthetic
cttgggggcaaagctgccctgaccctttcgggtgcgcagcctgaggatgaggctgagtattactgcttgctctcctatagtggtgctcgagtattcggcggagggaccaagctgaccgtcctaggggctgatgctgcaccaactgtatccatc

SEQ ID NO: 156 - DNA, 165 bp, synthetic construct
  source 1..165: mol_type = other DNA; note = synthetic
tcaggcctgaatcggtacctgaccatcaagaacatccaggaagaggatgagagtgactaccactgtggggcagaccatggcagtgggagcaacttcgtgtctgtgttcggaggaggcacccagctgaccgccctcggggctgatgctgcaccaactgtatccatc

SEQ ID NO: 157 - DNA, 164 bp, synthetic construct
  source 1..164: mol_type = other DNA; note = synthetic
tctggcacgtcagccaccctgggcatcaccggactccagactggggacgaggccgattattactgcggaacatgggatagcagcctgagtgctggccccgggtgttcggcggagggaccaagctgaccgtcctaggggctgatgctgcaccaactgtatccatc

SEQ ID NO: 158 - DNA, 22800 bp, synthetic construct
  source 1..22800: mol_type = other DNA; note = synthetic
aagctctaaaactacaaactgctgaaagatctaatgactaggacagcctagtaattttcataggggcataaatgtgaaacgccttgtgcatcgtagaagaaagcagaagagaaagcattcccaatttcttaactgccttttacctatattaatcagtaatatactggcttttacctctgttaatcataataaacaaattctcaataaattttatcgatactcttcaatgcctgctcagcaacattttccgaaggcagctcaagatattaaataactcataagggccaacctcctattgcagcattctttgggatttaaccagtttcccaagactcttttcacaatgttaagatgttagaaatagatccaaaactaggtgatatatcccctagtaaaactgtgaggtcaaacttgtctggctaatgcttccatttaaaaatttctctttcttgatccttcattgtatgtacacaataaatcaggggaaaactttaactgagtgaatcaaagtattctcattattataataggagcttcacacacacacaaaaaaatcaattctattactctcagcctcagttcctaaagccaagttaaagtcctgttctaagatcattgttgcatgaccatatgtattccaggtctaatctaaactgtggataaatcccagcaggacattagagatttttgtgagagtaagcatataggattcagggtttatgagctttagatttttcttgtcaaaatgaatgagagttgccatatctaaaaattattcccagataaataaaattcactacctagaattaatttatgcatataagtagaaatgctatctccctttttaccatccaaagtggaaagcctcatggaactagaaattaatattagaaaaatcagttaataaaagtatgtcatttcatcaattcaataagttataatagcaaaaaaccataataaattatcacttaaatgtcaatacatttataaactatggtacataaataggatattgaatagccattgatgctcctgatgaaaattagcaggcagtgataaatgataaatatgaagcacatgtcaataaataaaataagttttatgtaatttaggagaaaatggtgataatgacacaaaatgtgaattatggatgcatctataaaattctttgtacatttgtgaattgtaaatatttatcttagagacattattactttgtatatgttccatttgctcacctatatgtcccagtctccttacaaatgctatggccaaagaaataggcatacatacatcctttgcaggctgaggcaggaaaaagatcttacggaattttccagtctatcctttatctgtataagcaacttaagaggccatgtgctccaaatggtgcaaatacaagatggtagagcctctgtctgcctggatccttgagtggctgcatggagcagagcacctttctggccctggtgaagattgtagcatgagcaagatataagcatttgttggagctaggccatgagatttggggcagtggtataacctaccctattatggaaaatataaatacacaaaacagaaaagagagagagaagtgagagaagactgtgagagaagtgcatgagagaagactgtgttttgttcatttcctataatcctatatcaccatgggatcctgtgccttctggtgatcaaactaatgttctacagctccaaagaagaatgctcgcctaacgtctccattccaatgacctagagactaaaagccaaaaagaaccttagaaattatctattgcattctttgatgtaaggaaatatcttagagggcacagatagaaatatcttaacccaggtcacttagttcgtggcagagctgaggctaaaaccaggccttttgactcctaattttgtgctctttacaccttctcacatcacttctccaacccaaagtctagcagaaaaggctaaaataagatatatgcatagatttgctattataagtccatgtacttcctcagacgctttaagatggggcttctcatggttcacaataagcagcagagggaagtgaataactatcttcgtctcccctactgctatttgtgcagtttgaagcttatctcttaaatcatgttttcttctcgtagtaaatactacaacttgtgccttttatgtgtgtataaattttaatataatttttttccatgaaccattcaagtaaaatggacactccaaaaagatgttcaataaggttacatggcttcacattgccccctctacaccatcttgtggagctacacattcacctcacccaaatttgagaaaaataatcaagaaaatgactctcactagcagtgagaccaagtccataagcactaatgtcatcagtgcacactgcagcctcatgctgccaagcatgttttgggcgtatccctggactggtttggtgacatgatcaaaggtacattttccacctgcatagccccatcctggatctatagccttccttgtgtctttgtgaacaacctagtgtgaactcaaagtatgagacagatctcaattaatttagaaagtttattttcccaagattaaggacaagcccatgataaagcctccagaggtcctgatatatgtgcccaagggggtcggggcacagcttggtgttatacattttagggagacaagaaacatcaatcgatatgtagaagatgtgcatcgctttggtctggaaaggtgtgacaactcaaggcagggaagggggcttcctgctggggttgcattgttttgagtctctgatcagcctttcacatgtgaaaggcaggtagagaaatagtcatttatgccttagtctggcttattgaaacagtagggcagaagaagcattgcatatgcatttgtctgaagtgaacagagggatgactttgagctctgtcctttctttgtccacaaggaattaccttgtgggcaaattgtgagggaggtatgtagcttttttttctttgtagctatcttatttaggaataaaatgggaggcaggtttgcctgatgcaattcccagcttgactttcccttttggcttagtgatttttggggtcctgaggtttattttttctttcacattagtataactacttttctttttctaattccttttctacttgtatgtgttacagctgacttatgttacttgcaaaaagaattctgactaatgcaccatctgactagaaggcagggttcttcgatgataacgaatcctccagaatctagtaaacagaattgcctgaaaaagaggtgggtgtcttcttggggaatttctcatggcaatgaatggcaactggccaaaggatttatgaccagactgagctctcttttatctattctgttactcaccaagacctattagggtttgtgctccacagggacactggtttctaagttctagggttaaacagtccactcccaggcccaccacaccataccctcctgacatctggtgaacagcaataaaattgtttcttattctgaaaatcctccaatacttccaccatccccaaaaatgcagtggaggaggagagaaaatgaattgttccattagagaacacaatatccattatattattcttggcctttgagataccttacaaaacaaatacaaaaaaagtcccaatttaacatcttttaataatctttacaaaacagaacacatctcctttcttgataatagtcaagaggctcagtggcaactgtggtgaaaagtgtcagattctggtcatgtttcaaaggtagaaaaaatagaatttgttaacatattggatgtgaggcgtgggagaaacgtgaaatcaaggtggttgcaagtgtttaacctgagcaactagagaatttggaaggacattttctgagatggggaaggcaggcgggaatcagggattagagttgaacatattagacatttgagatgcctgctagacctctaattggcaatatcccttggacaggtggatgaatatgcgtgattctggagttcgggaaatagtccgggtggagatgcaaatttgggaaacagggcgaggttactagcaatgagttaaatcaatgaaggcaggctgggacctggcaggtaacccaacaagtagaggtcgaagagatgagaagaaaacagcacaggagacttagaagcagtggtcaggaggaaggagttgaaccaagaaagtgatgtcccagagccaacaaaataaggatttcttttctgtttacaaatgtaaaattaaaaggtttaataaaaagaaaatttacttttatggttggttgttattaagtggtccaaacactgtctcctatttgtagaatcagaactctctcatggcagtagaaaatttggaaagttactttttaaaaggtgtgtgcactgctgccctttgctggtcaagtttatgcactgcaaattccaaggacgattgctcgtcagcttttctcctttaaaatagctcaggctgtacaagctagaaagaacctcgcaagatattccttccaacatttgcatttgacttatgggaagtgcaggttcagccagaaaagttgtgtgcaaggccgtttatgtaagtttatcagacctgattcttacggctcttcccattgtttcgagcctcccttccattcacttcccgctcatacgcgaccaagtataggacaggagtagttattctgcactttatagcagctccactgtctggcactctgatgttctttaattacaagctttatgacagtgattctcaacctgctccactgcctccacctagtggcagaaagaagaaaatgtgtgtaactcgggagtctctggtctgaaagctccggggtatcatttcttcaaagtcttgagcttgtttttgtttgtatttatttatttatttgttttagagacaaggtctcgcactgcactccagcctgggagacagagcgagacaattcaggatctatctagtgaataaagagatatcagtaatgactgttttatattgtggctgtagcgcattcgagggataattcgattctgttctgctttcgaatgcatggctcactgtaacctccaactcccgggctcaagcgatcctcctacctcagcttctccagtagttgagcttgatttattttaaagtttcataaaattttggcatttctttccacaatatggccatgtgtgctttactataaaatattttcatcacaaaatttacatcgctggaaatccccataagccagtttgagaaacacaacccaagaaagcagaacagactcaaattatcccttaaatcccccttaaccacaaatataaaacagtccgtgactgggcgtgttggcttacacctgtaatcccagcactttgggaggccaaggcgggtggattacttgagctcaggagttcaagaccagcctggccaacatggtgaaaccccgtccctattaaaaatacaaaattattcaggagttgtggcaggcagttgtaatcccagctacttgggaggctgaggcaggagaatcacttgaacccaggaggtggaggttgtagtgagccaagattgtgccagtgcactccagcctgggcaacagagcgagacttccatcttaaaaaaaaaaaattaagtaaataaaatataaaaaaataaagcagtccctattgatatctctttattcactaaatcaacctggaattgacctgaattctgatttttttttcatcatggattttttgcattaattttgattgtttaaatattgcattaaaatattatttatcttgactactgagtttgcgggacctccttaaaatttatgaccaaggcaatgcctcactcactcgccttaccataatctgggccacatatcaggggctccaatagcaagcaacatgacttttgaacagctaagacttctctcttcactgtgaagaccagatgggccctgcaaacagtgtaacctctacatgaaaatgcacgagattccaactacaaccaggcacaaaagactctgatggtgaagtcccagccctccaagtcccaacttcctgaagggaaagagcaccccaagttctgaccagaggccagagtcataacgaagatggaatgtgagcttgacatagaaggggtggtagcacctggctcagtaatgaagaggctttcggtcctgaaggaagagctcagcacattcaaagattagaagggaggtcccagtcataggagcagggaaggagagaaggcccaataagaaacacagacaggagggaggggtcagggcaagatcatactggaaacaactagagagctaataaaagtcacagtgcccagtccccacatggaccagactcttcggaatctctaggcatcaatttgggcaccagtagttttcaaagttctccagaagattctatgcacaccagccaagggtgggaaccacaggtgttggcctagggatcatgacaatgagtttctaagtgcaataagaaacctccagagagtttaagcaggggaataatttgatttgtttcttgtttgtgatttttaaagatcagtctggttactgtgtgtaagacaataatccagaaaatctgttgctcatgaaccacatatctgtaaatttgcttcccctgtaactggatctaaccaacaaaaattagtacttactaagaaattacatgcccagggactatgctaagtaattcataaacactattttatttactcctcacagcaagtttataagagaaacgttattatttccacatttcggatgagaaatttgaggcttggggaaagttaagtaatttacctaatgtcacacccagttcataagatgcagagttaagattctaattctgtgtctaagttgatgctccatcaaacacaccacgcctccaactaggaagcaacatgctggccagaggatgctgtcatcaagtttacagaatggttagatttctaggcacagatgaataaatcaacatgttggtttgcaatagaatgaatctatccagctctgaatttgcatccaagggtttgtgagcacacaagtctaaaagtgtggcctcagctctgctaacttcatcaaggtgaatacctaggaggccaccctctgagaccaccagatggacagtccaccatctgtttacagatggtaaagccacataccagctttgccatctgatgttctctattcacattcaacatttatacaagaaatagtcatatggatccttttcaatagacagtactggggaaattgaattgccatatgcagaagaatggaactagacctctatctctcaccaaatacaaaagttaactcaagacagattaaagacttacatataagacctgtaactacaaaaacactagaagaaaacctagggaaaatgcttctggaattaatctaggtgaagaactcaggactaagatatcaaaagcacaagcaccaaaacaaaaatagacaaacaggacttaattaaactagaacgcttctgaacagcaagagaaataatcaatagagtgaacagataatctgcagaatgggtgaaaatatttgcaaactatgcatcctacagggaaataatgtccagaatttagaaggaactcaaacaattcaacaacaacagcaaaataaccccaccaaaaaagtgggcaaaggacatgaatagacatttttcaaaagaaggtatatgatatggtttggctctgtgtctccacccagatctcaccttaaattgtaataatccccacatatcatgggagagacccggtgggaggtaattgaatcatgggggcaggtttgtcccatgctgttctcatgatactgaataagtcctatgagatctgatgattttataaaggggagttcccctgcacacactctcttgcctgcctccatgtaatatgtgcctttgcttctcctttgccttctgccatgattgtgaggcctctccagccatatggaactgagtcaattaaaccactttttctttgtaaattacccaatcttgggtatgtctttattagcagcataagaacagactaatacagtgtacaaatggccaagaagcgtacaaaaaacaaaatgctcaaatcactaatcactagagaatcgcaagttaaaaccacaatgagatattatcttacagcagtcagaatgcctattattaaaacaccaaaaaataacatgttggcaaggatgcagagaaaagggaatacttacacattattagtgggaatgtaaactagtacagcttctgtggaaaacactatggagatttctcaaagaactagaaatagaactaccatgtggttcagcaataccacaactgggtatctacccaaagggaaataaattattatataaaaaagatatctgcactcacttgtttattgcagcactattcacaatagcaaagatatggaatcaacccaagtgtccatcaacagatgattggataaagaaaacgtggtgtgtgtgtgtgtgtgtgtgtgtgtgtatacacataccacaatgaaatactattcagctataaagaaaagaatgaaatcatgtcttttgcagcaatgtggttggaactggaggccattatcttaagtggataattcaaaaacagaaggtcaaatgtcacatgttctcacttataagtgggagctaaatgatgtgtacacatggacatagagtgtggtatgataaacactggagattgagatgggtggaagggtggaaggaggttgagtgatgagaaaatactaaatggatacaatatacatgattcaggcgatagatacactaaaagcccagacttcaccactacacagtatagctatgtagcaaaattgcacctgtattgcttaaatttatacaagtaaaaaaaagatcgtacgaattctgttttttattctctatgaaattactactgagagtattatccaatgccgtttctatgcagtgcccccaatattatccatttagcagctcctatgcaatgccccaagatagaaattgtcttcaacttttatcccaggaaaaccttcagtcacacgtagaaactagaaatttttcccctagatgaaagttatgtaacataacacattatcttcatttagtcggtttccaagaagctcagaaccagattttatgttcaatcaaaaactgcttattttaagtgaggtttactgaggtataaattacaataaaagccaccttttcgtgtatatttctataagttttggcaaatgcatagctgtgtaaccacaaccacattcaagatataggacaagtccctcatcctttaaagttcctttatgccccttccttcaccccagcccttggcaaccactggtttttgtctgatccaatcgtttgcctcttcctgaatgtcatgtaaatagagccatgcaatgtgaagccttttgagtctggctttgttcacttgttcacttaggagaatgcatttgagattcatctttgctgtttcgtgtagcactagttcactgtctattgttgagtagtattccattgtgtggatatgccacagattgtttatctagttaacaatttaaagccatttggtcatttctaatttttagctgctaagaataaagttgctgtaagctttccaatgcaggtttttgtgtgaactcaggatttcatttcgcttgggtaaattcctagctttgggactgctgagtcatctggtaggtgtatgttgaactttataagaaactgccaaactgttttccaaagttgctgtgctcttttgcactcccatcagcagtgaatgagggttccacttgctcgagcctagtattttaacttcactatataccttctttgatgacatatcctttcaaatttttggtcaagtttttattggggtgttgttactatggactgtgagagttctttgtatattctgcatatgatttttttctcacatttgtgttttatgaatatgttctcccaatgtgtggcgccttttattttcttaacgtgccatgtgaagagcagaagtttaattttatgatgtccaaattatctttttttcttttcttttttagatcaaaataggggtctattttgattaccactgttattttatctccatttgattttcgatttttatttttatttttctaatttcattgtaaatttttaattaaacccaaatattctaggggaaagaggcaagataaaaatagtctaacttgggcataaattttagagtcatattctcttgccgagaaaggaaactagctctcttacattgattgtttaatttcagacgtcactactttatgaggatgcccaaattatgggctttaaaaaatatatatccaaacaggggttcagaaagaataactaatttgtccacaacaacacaaaaaatgattccaccataagtttgcccagtgacagggtctatattattttctatatatcaaattctacaactggttcttaaagctactgtacataacctaagttaaaatattaggtattagttgataagacattttatcatctatgaaatgttgcctgttgtcatagttagagaatcttttaaaatatggagctattttcatagattaaactatgccagttaaaagttgggtaaaaagaactacagaataatatttatgtttatcgtgtaaggttttaaagcaaactccaagtcattttcatcaatgaaatcaataaggttttgcaaatatatatgtatgaaaatactgatttaaaatgcaaataaggggagagtttgagagagagagagagaccaaatgattttataattctagtaagtttataggtttatggggtttttacgtacttttctacccaacttgtctataagactttaatgaatcacttagaatttttaaaataatttattattactctgtacctgttctttactctgcaaatcttaccttgcccttttgtctaaaagcaataaaatctgacctggtttatatcgtatcattgattttgttacttagcaagcacagtgatccattaggcctatgtaggctcatggtttatacaacactgccatctgctgacagagtgtgacagtcacagtcagcaacacgagaccactttattttcatttttagtgtttatagaaatatgaatatacacaaatagtataatgaaccctaagcttcacaaattaacattttgctaatcttgtttcaactaccgcctcccccctcatccaattactctgttctctcacctcctcacacacagacactggcagtatttttcagccaatcattaatacgttgccaactgataaggacttttaaaaaacaaccaccattccattatgattcccagcataattgagagtaattccctaatatccaatacccattttctattccaatttccttgattgtctttaaactgtttttaccctaagtttgcttaaatcaaagtccaggtcctgttaaacatatggttaagttttacccaaacccaaataaataaataaataaataaataaataacctattttttccaattccagggaatagtgaaagagggtaaatgccattatttagaaacataaatcacatcataggactagaattatcttgaagtcaaaattgaagactgaaaatggaaaagaaaggtatagactaaacttatttaaaaacttcaatgcagaactctaagagaagatattagaaagttgtaccagcattcattattcagtattcatcagtattcactcagctatatgtagttgaaatctaactagaggagcttgatcagataaagagatacatttttctcaccaaggcggactctggaggcaggtggttcagagctagacagctgctgcaggacccaggtcctttccctgcctgctcctccactctagcttgtgactttcatcctgcaagatgggtgtttctgccaagttccagatagaagaagatagaacacaaaggagaaataagcagtggtgcctctgtccatcaagcaaaatttttccagaaatgcacaatagatttcagatgatgtctcaacagtcctaactgcaaagaagctgaggaattagatttttggctgggacactgttgccctgtaaaaaaattgggattctgttattaaagaataagaggagggaagaaagattgaaaactcctatgcaatagtgaaaaaaataagaaactcaataaaaaagtgggcataccttaaaaacaggcaattcacaacagatgagaccccaatagccaataaacatttttaaatggtcaacctcatgagtgatcagaaaacacaaatatgtattttaaaccaaaaataaaatacaatgtattgaccatttgagtggaaaaaaattaaaaagcctgataatatcaagtattggagaggatgtagagtgaggaaactccatggaggacctatcattgcaaatgtgggaatgaaacttaatacacgaatttgaggccaatttgtaaattgaaaaatgcgcacaccctgcaaccaagtaccccttgcaatatttttgaaaagacaaaaacgttatgtaaatggaatcatgcaatatgtgacctttatactcagcataatgcccctcagatccattgaagtcatgtgtatcaacagctcactattttttttttaattttttttagagacagagtctcactctgtcacacagggtggagtgcagtggcgagatcataactctctctagcagcctcgaactcctgggctcaagcatcctcctgcctcagcctcccaagtagctaggactacaggcatgggacacaacacacagctaatttttttaaattttttttagagacatggtctcactatgttgcctacgctggtctcaaactcctaggtcaagcgattctcccacctctacttcacaaagtgctgtaggtatgtaggtatggattgtaggtatgaaccaccgtgcccaactcactactttttattactaattattccatgggatggatgtaccgcagtttgttttaccattaatctattgtaggacattttgactgattccagtttttttttaatacaaataaaaccactatgaatagttgtgtattgtatacgtttttgtgctaagttttcatttttctgggataagttttcatttctttgggcttttactgtatccttgatattataatatgttacatcttcagttttattctattcaatatataatcttttattttccttgaaatctcccatggattgtttagaagtgtgttgttttgtttccaagggtttggcatttttcccattatttttctattatcgatttccagtttgattccaggtggtcagagaacacacttcatgtgatttcagttctattaaatttgttgaggtttgttacatggcccagtatatggcaattttggtatatgttccatgagcacttgaaaagaatgcgaattctgctggtgctggttggagttttccagcaatgttgatttatgatcttactcattgatggtggtgttgagtttgatgtgttcttacgatggcagctttaacattcttgtcaggtaattctaacgtctctgtcatgtcagtattagcgcctcttaactgtctcatcaaagctgagattttcctggttcccctggttcctgttgggatgtgtggttttcatttgaaatctggactttggagtattgtgttatgaggctttggatctcatttaaactcatctcagcgaatttcctctcttgccactcaggaaggagaagttgggtgtttgaatggagcagagccgttactgcctaagaattgttttactgggcttcccctttctttctcctttgactagagagagccagctttttattagggctttatgtttttctgggcctgttggtgtttctgggttgacaaacttctccagaaccaagtctggaatggatgaggcaaaaagaaaccccgtggaatgcactgctgggtcgctccttgggtcccaatgttcctaactggtctgccttcttctctccagcttccagagtcttcataagtttgctttacgtacaatgtccggggtttttactttacttgagagaaataggtaaaagtaattctactccatctttcaggaagcaaaagcccccttgtgtatttttttaaactttcaaaaacaaaacaaaaggcagctgcaacagtaaagaagctagtaacacccttggtgggaaattcaagtccaaatacacattttaagtttggctagccagtgagaacatcagaatagttcaggttttaaacaaatttatatttatgattatgcatatactaaaagctgaaggcatcttatatttactaagcacctattttgttcttgttaaaaagacagaattccattccctaggaaatttgacctggcagctggagctgatccacctggccactagagcacagagcagggagagtagtagccctgccccagccacccctcaagacaggattctttctctgggaactgtaggtaacactaaatcgttctggaacacaacaacgaaagaagaaaggaaagagaaagaaagaaaggaagaaagagagagagaaggaaggaagggagggagggaaggaaggaaggggaagggaagggaatggaagggaaggaaggaaggaaaaggaaggaagggagggagagagggaggaaggaaggaaaggaaaggaaggaaggaagaaggaaagaaaaaaagaaagaaagaagaaagaaagaaagacaagaaagaaagaaagaaagaaagaaaggggaaagaaaagaaagaggaaagaaagagaaagaaagaaaagaaagaaaggaaagaaagagaaagaaagaaaaagaaagagaaagaaagagaaagacaagaaagaaaaaggaaagaaaagaaagagaaagaaaagaaagaaaggaaagaaagagaaagaaagaaaaagaaagaaagaaaagaagaaagagaaagaaagaaagaaaaagaaagaaagaaagaaagaaagaaaaagaaaaagaaaggagaaaatgacagcaattacttttgcaacaacctaatataagttttttaaaagttaaatattctgttccatgcattgctggataccttataaataacagggcatcctatgacctgaatttcccaaattatgagttgagggtttgaactagttttaaaaaacaaggaggccaggcgcactggctcatgcctgtaatcccagcactttgggaggctgaggcaggtggatcacgaggtcaggagctcgagaccagccttaccaacatagtgaaacaccgcctctactaaaaatacaaaaattagccgggcgtgatggtgcgcacctgtaatctcagctactcagcaggctgaggcaggagaatcgcttgaacccagaaggcggaggttgcagtgagccaagatcacagcattgcactccagcctgggcgacagagggagactccgtcttcaaaaaaaaaaaaaaagacaaggaatctgtaaaacaggcactggaagtatatgcacttttattttcattctatgctatccgatgcctactgctatttcccttcatatttaacctccaacagctgcattttgctccctccagaccacctgattggagctcacgtgctcccacacagtacctccaaccagagagagtcgagtcccacagaaaggcgtaacaatcaccagtaattttgcacttattttacattgtgccttgatacagagtactcaatgaatgctctttgaatcatatttaataaatatgtgtatttgggattgtagcatattgcagctacctggatatataatttaattagaaaaaaaattttgtgtggctcaatcaacaaacgacttttctctctctctctttctctttctccctctctctctctttcttctcagttgatgttgctggagttcagtgttgtgcagatggcagtgacaaatgccatgggcacatgagatatgataaaaggtccctgaagaaggtggagaaccagttatcttatgaaattttccagagtgggtactggatctctcctgtctggcaccatgctggcctcagcccaaggggaatttccttccagagacagagggcagtgattgaggtggggagacagatcgtaacactgagacttacatgaggacaccaaacagaaaaaaggtggcaagtatagaaaattctttcttctggacagtcttctctgttctaacttcagcaaaattctccccccagtggatgctattgcacaaccctacatatgctatgttttttcctatacacacttacctatgataaaatgcattaattagtcacagtaagaggttaacaacaataactagtaataaaatagaacaattcagtaaaataagagttacttgagcacaaacactaggatatcatgacagtcaatctgatgaccaagagggctactaagcatctaaacaggagggtaagtgtagacagcatggagacgctggacaaagggatgattcagtcccaggctggtatggagcggaagggcatgatatgtcatcacgctactaaggcacacaatttaaaatgagtaaattcttatttctagaaatttctttttaatattttcagactacagttgcctacaggtaactgaaaccccagaaagcaaaattgttgataaggaggtactactgtacatcgtcctttgaaccaactttatcatttgctagtatatacatatatacctacatacatacatatacacatacctgcacacacctatatgtatacgtacacacacacacacgcacacacacacactcacatctactaatgttagaataagtttgctaaataagatgcacaacttgttaatgtcctacagagcaataaaaccataagcattggggttatcttttctactagataaaaatccattatcattttcataaagttttctttacattaacatctaacttttgcaatctagtttttaatcatcataaataggaagcaaatgaactgtttctctagtgaatcaaatatccttgaaaacatacatagtcatctttttggtttatttttatttttagataaattatttaaagttttaaataatttaacattcacaatagtttgtgactgtatattttgacttggtccttcaaacttaatttgtacttttatgtatcgtgcttacctcaattttttattcacttttcctaaactttgctggattggtttattatttttgtctatttcttttccttctagtggtttgggagggttttttaaatcccattactattgaatgcctattaacttgccccctttttctttcaatctctattcccacggcctgaagcatgagggccaagctgtctgtaaccagcagagagatgacccaggtgttattccactctccactgtccacctatcaccattcccagcccgatagctctgaagtacggcttttctggggctctgtggggaaaactagaactggctgcttcaaggacacctcctgtttttgcaatggaaaaaatgtttctaaattccagtttctctatgaattcaatgacatggtttaaatctctgtggtgttcttcaaagttttttcttctaataggacctctcatgattctccaaccacgaaataaattcattatcatttttatatttcttctgtcattgcaaaggaggttttgaaagagtggaggacgcgctaatgaactcaaaaatccacactattccttgtttccatctgttgttcattcattgtttccattggcctgtccgcctcctatcctccttcttagacttggagctctagcctcagccaggatagggaaaagagagatcagactgttactttgtctatgtagaaaaggaagacataagaaactccattttgatctgtatcctgaacaattgttttgccttgagatgctgttaatctgtaactttagccccaaccttgtgctcacagaaacatgtgttgtatggaatcaagatttaagggatctagggctgtgcagaatgtgccttgttaacaacatgtttacaggcagtatgcttggtaaaagtcatcgccattctccattctcgattaactaggggcacagtgcactgcggaaagccgcagggacctctgcccaggaaaactgggtattgtccaaggtttctccccactgagacagcctgagatatggccttgcgggatgggaaagatctgaccgtcccccagcctgacacccgtgaagggtctgcgctgaggaggattagtaaaagaggaaggcctcttgcggttgagataagaggaagccctctgtctcctgcatgcccctgggaacggcatgtctcagtgtaaaacctgattgtacattcgttctattctgagataggagaaaaccgctctgtggctggaggcgagatatgctggcggcaatgctgctctgttgttctttactacactgagatgtttgggtgagagaagcataaatctggcctacgtgcacatccaggcatagtaccttcccttgaatttacttgtgacacagattcctttgctcacatgttttcttgctgaccttctccccactatcaccctgttctcctgccgcattccccttgctgaggtagtgaaaatagtaatcaataaatactgagggaactcagagaccggtgccagcgcgggtcctccgtatgctgagtgacggtcccttgggcccactgttccttctctatactttgtctctgtgtcttatttcttttctcagtctctcgtcccacctgacgagaaatacccacaggtgtggaggggctggacaccccttcgagccaggattatcagggcatttgggggtctgcaaaactaagccccaactcatcgatttcacaacttcatccagagccagcctgaacagtagttgcccatgatttctatgccttaatacgagaagagaacataggggctgggtgccaagtaggtagacagggagggcagggaactctaagacagagcttgaggggctcattcctcttgcaaaatgaaacaaaaaccacagcactgaatatgtaaatctcggtggctgaacccctcctaggatagtaagccctgacacaattgctgctatcttctctttctctcaaggaagtcaaaaaacacctgcagccttactgtccccttggaaacaagatgaacatctacattttctaaagtgggacaagaatctctgttcatatttatgtcccatgcatttgcacgtggccggacaaaggactttgcttctgccagcacatctgtcttcagatatgagaggaaacagacacaacctggaggcggcaaagaagcagctctttctcaagtgacctcctctatctccctacttcctggctaatggggcagccttgatccttgggaatccaggacagatatccactcgtgacaaactagctggaagaatgacaaccaatcaggttccaagcaccactggatgtgaaccacagaatttcctcctctccttgtggaatgtcagcttacgtctgacaaaaaatgtaaaactgagagagttacaatcttaaggaggagtcaagctaaagcagaaagaatcacctactctggactccagcatgactgctgagctcaaatatatatagagagagaaagaaccacaaacttgaagatggatatcagctacagactttcctgagtcaggtagggaaatggccatccctcaaaccttgcaaaaggcaaacttatgccattgtgtcctctgacatactgggtgatgtactgtatgttactgatgtgaggggaacttcctaaattggctagtaaattatgccaaataaaaagcaaaaatgatatttcttgaaatgttacatctgaggaacattgctaaaataatttatcagtagttttcaggatgatttatagatgtgcattgaagtgtgtacttgtgctctctctctcctctctctctctctttctctcctctctctcgctctttctctccttgcccccctccctccctgactttccttcctgtcccctccacagcagtttatattttttttctgataatctaactttgctgagggttcaatgtaaagcaccttcagtgatgagttagttggaatgttccccaagaaattctatttccagcactcttttacatgaaatccaagaagctctcagactatcttactgacaccttgcctttcctcaacagatcaatcttatcaatgtccatcacagatattttgtagaacggtggatcctggcagagtctcacagatgcttctgagacaacatttgctttcaaaaaatgaaccacacacatcctaaagatctcagccacttcccatgtttcattttgtgttacagcaaacatcacaacaatcattcctacagatcaccactgcatgtgatcaataaaatagtttttgcaacaatggtacttatgataatcatcttttattgtttacaaatactgctttacaatagttattcggttgcactgttcatattagatttccaattagctcacttaggaacataagtccctcgaacagctcagtcatctttttcattcctgtttctatcccctacatctctttcctttgcagacgactatctcctacactgaaacaggaaagcttttacctttttggcatgcttgatttaaagattatagaaaagtatttgacaaagaaaactcacacatgtgtgtacatatcttttaaaaagttatgtttatgcattgcacaggaatatcgagaatgctaataggcaatgtcagagtttactgtttttcaaaattagtacagttttattatttctaaaaactataaaatgaatatattcacatcaccatacagaagagtaggaggagatggcataaagtgtcattgttcctcctctgcaatcccaggagataactaccaagcacaatttatgtcttttaaaattcagcccgtatttatatacatatatattcaatgtagatgggatcatgatatctcaccacacatactcttcagtgacctgcattttcacaaacaccttccacgtaactatatagaagtctacgtcttccccttaatgtctgctttgtgctacattgtaaagctctagcacagtttaaccaaactcctattaatgaggattttagttatttttcactctttaaacaatatttccatgtgtagtcttatacatacgtctgtacacacttatcccagtctaaggagttccttttaccttcccccatcccagcattccctgtcacgcttgttgcttccgttgagtgactttactcctggagtataatctgcgtatagttcagttaaaaacatgggatctgagtttaggtcacagctctgccacttactgccataagccagttccttgacctctctgccctcaagtttttgcacctacaaagtaggggataatattagttcctagttcatagagtcttgggaataattaaatgtgatgatccatgtacaatgtctggcacttagtaagtgctcaataaatgtcaccctttatgattggtattgcgtgtatgtctgcagagaaaatcactttgtgtcccctttaaaaaaggactatgcccttggtcagctattttgcacattaaatttcacttgccaatattaactctccacctctaacttgatccctctccttcctcatcttctggtgagaccaaatgctaattctgctattcaaggcaactagcaaagctgccagtgacagaatcaaataaacctacccctaatctttagaattgtagttatgatttctgttgtaaaagttactgttgtggcagtcagtattagtctttggtctatgatagcatctctgatctattattgaytttcaattakgtatttttttttatttattctgaaaatgtttgttaagcatttgctaagtaaagatactggackgagcctcccaaatacagggcaaataaaacatcaaacagcttataatttagaagggtagaagagaatctgaaagcaggtaaaaataaacaggcactcggctgggcgcggtggctcacgcctgtaatcccagcactttgggaggccgaggtgggcggatcacgaggtcaggagatcgagaccatcctggctaacacggtgaaaccccgtctctactaaaaatacaaaaaattagcgaggcgtggtggcgggcgcctttagtcccagctagtcgggaggctgaggcaggagaatggtgtgaacccgggaggcggagcttgcagtgagccaagatcgcaccactgcactccagcctgggygacagagcgagactccgtctcaaaaaaaataaataaataaaataaaaaataattaggtactctaggcccagtgacctgtctctgtactctgtaaattcaggtcacctgctcagggctaatctgagagaaggtctctcttcagttgaattttgaaagacaattagcagttcacaagctaacccaggtggacaaagatgttcccaagcagagggagtgcttgtgaaagctggaggccatagaaaaactctaaggagtgtagggaggtgggagtaatgtatggaaggggtggagatggaaggttaagagagatacaaggctgcaaaaatggagctggactcaaaagaaaatactgaaaaggtcttcagtgttgttgatgagattactatggaaacactatggaacactgggactccatggcagctccaaagatggcatgcgcctggtccagctcagtaagagctgagctcttcctgtg

SEQ ID NO: 159 - DNA, 154 bp, synthetic construct
  source 1..154: mol_type = other DNA; note = synthetic
tctggcaacacggcctccctgaccgtctctgggctccaggctgaggatgaggctgattattactgcagctcatatgcaggcagcaacaatttaagtcttcggaactgggaccaaggtcaccgtcctaggtcagcccaagtccactcccactctc

SEQ ID NO: 160 - DNA, 156 bp, synthetic construct
  source 1..156: mol_type = other DNA; note = synthetic
tcagggacaatggccaccttgactatcagtggggcccaggtggaggatgaagctgactactactgttactcaacagacagcagtggtaatcattatgtcttcggaactgggaccaaggtcaccgtcctaggtcagcccaagtccactcccactctc

SEQ ID NO: 161 - DNA, 150 bp, synthetic construct
  source 1..150: mol_type = other DNA; note = synthetic
tctgggaacacagccactctgaccatcagcgggacccaggctatggatgaggctgactattactgtcaggcgtgggacagcagcactgccgtcttcggaactgggaccaaggtcaccgtcctaggtcagcccaagtccactcccactctc

SEQ ID NO: 162 - DNA, 21 bp, synthetic construct
  source 1..21: mol_type = other DNA; note = synthetic
aggtggaaacacggtgagagt

SEQ ID NO: 163 - DNA, 21 bp, synthetic construct
  source 1..21: mol_type = other DNA; note = synthetic
ccactcggggaaaagttggaa

SEQ ID NO: 164 - DNA, 20 bp, synthetic construct
  source 1..20: mol_type = other DNA
ggtatagtgggagctactac

SEQ ID NO: 165 - DNA, 17 bp, synthetic construct
  source 1..17: mol_type = other DNA
ggtataactggaactac

SEQ ID NO: 166 - DNA, 31 bp, synthetic construct
  source 1..31: mol_type = other DNA
gtattactatggttcggggagttattataac

SEQ ID NO: 167 - DNA, 18 bp, synthetic construct
  source 1..18: mol_type = other DNA
gagtatagcagctcgtcc

SEQ ID NO: 168 - DNA, 11 bp, synthetic construct
  source 1..11: mol_type = other DNA
ctaactgggga

SEQ ID NO: 169 - DNA, 77 bp, synthetic construct
  source 1..77: mol_type = other DNA
gcaacaatttcgtcttcggaactgggaccaaggtcaccgtcctaggggctgatgctgcaccaactgtatccatcttc

SEQ ID NO: 170 - DNA, 77 bp, synthetic construct
  source 1..77: mol_type = other DNA
gcaacaattatgtcttcggaactgggaccaaggtcaccgtcctaggggctgatgctgcaccaactgtatccatcttc

SEQ ID NO: 171 - DNA, 74 bp, synthetic construct
  source 1..74: mol_type = other DNA
gcaacaatgtcttcggaactgggaccaaggtcaccgtcctaggggctgatgctgcaccaactgtatccatcttc

SEQ ID NO: 172 - DNA, 78 bp, synthetic construct
  source 1..78: mol_type = other DNA
gcaacaatttatgtcttcggaactgggaccaaggtcaccgtcctaggggctgatgctgcaccaactgtatccatcttc

SEQ ID NO: 173 - DNA, 78 bp, synthetic construct
  source 1..78: mol_type = other DNA
caagtcggttgtgtcttcggaactgggaccaaggtcaccgtcctaggggctgatgctgcaccaactgtatccatcttc

SEQ ID NO: 174 - DNA, 77 bp, synthetic construct
  source 1..77: mol_type = other DNA
tgagtgcttatgtcttcggaactgggaccaaggtcaccgtcctaggggctgatgctgcaccaactgtatccatcttc

SEQ ID NO: 175 - DNA, 77 bp, synthetic construct
  source 1..77: mol_type = other DNA
tgagtgcggctttttttggaactgggaccaaggtcaccgtcctaggggctgatgctgcaccaactgtatccatcttc

SEQ ID NO: 176 - DNA, 78 bp, synthetic construct
  source 1..78: mol_type = other DNA
ctgaatggttatgtcttcggaactgggaccaaggtcaccgtcctaggggctgatgctgcaccaactgtatccatcttc

SEQ ID NO: 177 - DNA, 78 bp, synthetic construct
  source 1..78: mol_type = other DNA
agtggtaatcatgtcttcggaactgggaccaaggtcaccgtcctaggggctgatgctgcaccaactgtatccatcttc

SEQ ID NO: 178 - DNA, 78 bp, synthetic construct
  source 1..78: mol_type = other DNA
agtggtgcttatgtcttcggaactgggaccaaggtcaccgtcctaggggctgatgctgcaccaactgtatccatcttc

SEQ ID NO: 179 - DNA, 78 bp, synthetic construct
  source 1..78: mol_type = other DNA
agcagcacttatgtcttcggaactgggaccaaggtcaccgtcctaggggctgatgctgcaccaactgtatccatcttc

SEQ ID NO: 180 - DNA, 69 bp, synthetic construct
  source 1..69: mol_type = other DNA
agcagcgcttatgtcttcggaactgggaccaaggtcaccgtcctaggggctgatgctgcaccaactgta

SEQ ID NO: 181 - DNA, 72 bp, synthetic construct
  source 1..72: mol_type = other DNA
ggtggtgcttatgtcttcggaactgggaccaaggtcaccgtcctaggggctgatgctgcaccaactgtatcc

SEQ ID NO: 182 - DNA, 75 bp, synthetic construct
  source 1..75: mol_type = other DNA
agtagcacttatgtcttcggaactgggaccaaggtcaccgtcctaggggctgatgctgcaccaactgtatccatc

SEQ ID NO: 183 - DNA, 63 bp, synthetic construct
  source 1..63: mol_type = other DNA
agcagcacttatgtcttcggaactgggaccaaggtcaccggcctgggggctgatgctgcacca

SEQ ID NO: 184 - protein, 21 aa, synthetic construct
FGTGTKVTVLGADAAPTVSIF

SEQ ID NO: 185 - DNA, 79 bp, synthetic construct
  source 1..79: mol_type = other DNA
cagcctgagtggttctgtgttcggaggaggcacccggctgaccgccctcggggctgatgctgcaccaactgtatccatc

SEQ ID NO: 186 - DNA, 79 bp, synthetic construct
  source 1..79: mol_type = other DNA
cagcctgagtggttatgtcttcggaactgggaccaaggtcaccgtcctaggggctgatgctgcaccaactgtatccatc

SEQ ID NO: 187 - DNA, 79 bp, synthetic construct
  source 1..79: mol_type = other DNA
cagcctgaatggtgctgtgttcggaggaggcacccagctgaccgccctcggggctgatgctgcaccaactgtatccatc

SEQ ID NO: 188 - DNA, 79 bp, synthetic construct
  source 1..79: mol_type = other DNA
cagcctgagtggtcgggtgttcggcggagggaccaagctgaccgtcctaggggctgatgctgcaccaactgtatccatc

SEQ ID NO: 189 - DNA, 76 bp, synthetic construct
  source 1..76: mol_type = other DNA
cagcagcactgctgtgttcggaggaggcacccagctgaccgccctcggggctgatgctgcaccaactgtatccatc

SEQ ID NO: 190 - DNA, 79 bp, synthetic construct
  source 1..79: mol_type = other DNA
cagcagtggtaatgctgtgttcggaggaggcacccagctgaccgccctcggggctgatgctgcaccaactgtatccatc

SEQ ID NO: 191 - DNA, 82 bp, synthetic construct
  source 1..82: mol_type = other DNA
cagcagtggtaatcatagggtgttcggcggagggaccaagctgaccgtcctaggggctgatgctgcaccaactgtatccatc

SEQ ID NO: 192 - DNA, 76 bp, synthetic construct
  source 1..76: mol_type = other DNA
cagcagcgctgtggtattcggcggagggaccaagctgaccgtcctaggggctgatgctgcaccaactgtatccatc

SEQ ID NO: 193 - DNA, 82 bp, synthetic construct
  source 1..82: mol_type = other DNA
ctactatggtggtgctcgggtgttcggcggagggaccaagctgaccgtcctaggggctgatgctgcaccaactgtatccatc

SEQ ID NO: 194 - DNA, 82 bp, synthetic construct
  source 1..82: mol_type = other DNA
ctcctatagtggtgctcgagtattcggcggagggaccaagctgaccgtcctaggggctgatgctgcaccaactgtatccatc

SEQ ID NO: 195 - DNA, 79 bp, synthetic construct
  source 1..79: mol_type = other DNA
gagcaacttcgtgtctgtgttcggaggaggcacccagctgaccgccctcggggctgatgctgcaccaactgtatccatc

SEQ ID NO: 196 - protein, 20 aa, synthetic construct
FGGGTKLTVLGADAAPTVSI

SEQ ID NO: 197 - DNA, 79 bp, synthetic construct
  source 1..79: mol_type = other DNA
gcaggcagcaacaatttaagtcttcggaactgggaccaaggtcaccgtcctaggtcagcccaagtccactcccactctc

SEQ ID NO: 198 - DNA, 81 bp, synthetic construct
  source 1..81: mol_type = other DNA
gacagcagtggtaatcattatgtcttcggaactgggaccaaggtcaccgtcctaggtcagcccaagtccactcccactctc

SEQ ID NO: 199 - DNA, 75 bp, synthetic construct
  source 1..75: mol_type = other DNA
gacagcagcactgccgtcttcggaactgggaccaaggtcaccgtcctaggtcagcccaagtccactcccactctc

SEQ ID NO: 200 - protein, 19 aa, synthetic construct
FGTGTKVTVLGQPKSTPTL